European Patent Specification EP 3 337 816 B1, published February 14, 2024. Title: Albumin variants and conjugates. Applicant: Novozymes Biopharma DK A/S. The sequence listing filed with the application follows.

SEQUENCE LISTING (152 sequences)

SEQ ID NO: 1 - DNA, 1761 bp, Homo sapiens
gacgctcacaagtccgaagtcgctcacagattcaaggacttgggtgaagaaaacttcaaggctttggtcttgatcgctttcgctcaatacttgcaacaatgtccattcgaagatcacgtcaagttggtcaacgaagttaccgaattcgctaagacttgtgttgctgacgaatccgcggaaaactgtgacaagtccttgcacaccttgttcggtgataagttgtgtactgttgctaccttgagagaaacctacggtgaaatggctgactgttgtgctaagcaagaaccagaaagaaacgaatgtttcttgcaacacaaggacgacaacccaaacttgccaagattggttagaccagaagttgacgtcatgtgtactgctttccacgacaacgaagaaaccttcttgaagaagtacttgtacgaaattgctagaagacacccatacttctacgctccagaattgttgttcttcgctaagagatacaaggctgctttcaccgaatgttgtcaagctgctgataaggctgcttgtttgttgccaaagttggatgaattgagagacgaaggtaaggctagctccgcaaagcaaagattgaagtgtgcttccttgcaaaagttcggtgaaagagctttcaaggcttgggctgtcgctagattgtctcaaagattcccaaaggctgaattcgctgaagtttctaagttggttactgacttgactaaggttcacactgaatgttgtcacggtgacttgttggaatgtgctgatgacagagctgacttggctaagtacatctgtgaaaaccaagactctatctcttccaagttgaaggaatgttgtgaaaagccattgttggaaaagtctcactgtattgctgaagttgaaaacgatgaaatgccagctgacttgccatctttggctgctgacttcgttgaatctaaggacgtttgtaagaactacgctgaagctaaggacgtcttcttgggtatgttcttgtacgaatacgctagaagacacccagactactccgttgtcttgttgttgagattggctaagacctacgaaactaccctcgagaagtgttgtgctgctgctgacccacacgaatgttacgctaaggttttcgatgaattcaagccattggtcgaagaaccacaaaacttgatcaagcaaaactgtgaattgttcgaacaattgggtgaatacaagttccaaaacgctttgttggttagatacactaagaaggtcccacaagtctccaccccaactttggttgaagtctctagaaacttgggtaaggtcggttctaagtgttgtaagcacccagaagctaagagaatgccatgtgctgaagattacttgtccgtcgttttgaaccaattgtgtgttttgcacgaaaagaccccagtctctgatagagtcaccaagtgttgtactgaatctttggttaacagaagaccatgtttctctgctttggaagtcgacgaaacttacgttccaaaggaattcaacgctgaaactttcaccttccacgctgatatctgtaccttgtccgaaaaggaaagacaaattaagaagcaaactgctttggttgaattggtcaagcacaagccaaaggctactaaggaacaattgaaggctgtcatggatgatttcgctgctttcgttgaaaagtgttgtaaggctgatgataaggaaacttgtttcgctgaagaaggtaagaagttggtcgctgcttcccaagctgccttaggtttgtaataa

SEQ ID NO: 2 - protein, 585 aa, Homo sapiens [sequence omitted]

SEQ ID NO: 3 - protein, 609 aa, Homo sapiens [sequence omitted]

SEQ ID NO: 4 - protein, 621 aa, Pan troglodytes
MNESSCCSTSLPAFGVSVLDSGHSSSSAYSRGVFRRDAHKSEVAHRFKDLGEENFKALVLVAFAQYLQQCPFEDHVKLVNEVTEFAKTCVADESAENCDKSLHTLFGDKLCTVATLREKYGEMADCCAKQEPERNECFLQHKDDNPNLPRLVRPEVDVMCTAFHDNEGTFLKKYLYEVARRHPYFYAPELLFFAERYKAAFTECCQAADKAACLLPKLDELRDEGKASSAKQRLKCASLQKFGERAFKAWAVARLSQRFPKAEFAEVSKLVTDLTKVHTECCHGDLLECADDRADLAKYICENQDSISSKLKECCEKPLLEKSHCLAEVENDEMPADLPSLAADFVESKEVCKNYAEAKDVFLGMFLYEYARRHPDYSVVLLLRLAKTYETTLEKCCAAADPHECYAKVFDEFKPLVEEPQNLIKQNCELFEQLGEYKFQNALLVRYTKKVPQVSTPTLVEVSRNLGKVGSKCCKHPEAKRMPCAEDYLSVVLNQLCVLHEKTPVSDRVTKCCTESLVNRRPCFSALEVDETYVPKEFNAETFTFHADICTLSEKERQIKKQTALVELVKHKPKATKEQLKAVMDDFAAFVEKCCKADDKETCFAEEGKKLVAASQAALGL

SEQ ID NO: 5 - protein, 608 aa, Macaca mulatta
MKWVTFISLLFLFSSAYSRGVFRRDTHKSEVAHRFKDLGEEHFKGLVLVAFSQYLQQCPFEEHVKLVNEVTEFAKTCVADESAENCDKSLHTLFGDKLCTVATLRETYGEMADCCAKQEPERNECFLQHKDDNPNLPPLVRPEVDVMCTAFHDNEATFLKKYLYEVARRHPYFYAPELLFFAARYKAAFAECCQAADKAACLLPKLDELRDEGKASSAKQRLKCASLQKFGDRAFKAWAVARLSQKFPKAEFAEVSKLVTDLTKVHTECCHGDLLECADDRADLAKYMCENQDSISSKLKECCDKPLLEKSHCLAEVENDEMPADLPSLAADYVESKDVCKNYAEAKDVFLGMFLYEYARRHPDYSVMLLLRLAKAYEATLEKCCAAADPHECYAKVFDEFQPLVEEPQNLVKQNCELFEQLGEYKFQNALLVRYTKKVPQVSTPTLVEVSRNLGKVGAKCCKLPEAKRMPCAEDYLSVVLNRLCVLHEKTPVSEKVTKCCTESLVNRRPCFSALELDEAYVPKAFNAETFTFHADMCTLSEKEKQVKKQTALVELVKHKPKATKEQLKGVMDNFAAFVEKCCKADDKEACFAEEGPKFVAASQAALA

SEQ ID NO: 6 - protein, 608 aa, Mesocricetus auratus
MKWVTFLLLLFVSDSAFSRGLFRRDAHKSEIAHRFKDLGEQHFKGLVLIAFSQFLQKCPYEEHVKLVNEVTDFAKTCVADESAENCDKSLHTLFGDKLCAIPTLRDSYGELADCCAKKEPERNECFLKHKDDHPNLPPFVRPDAEAMCTSFQENAVTFMGHYLHEVARRHPYFYAPELLYYAEKYSAIMTECCGEADKAACITPKLDALKEKALASSVNQRLKCSSLQRFGQRAFKAWAVARMSQKFPKADFAEITKLATDLTKLTEECCHGDLLECADDRAELAKYMCENQASISSKLQACCDKPVLKKSHCLSEVENDDLPADLPSLAADFVEDKEVCKNYAEAKDVFLGTFLYEYARRHPDYSVALLLRLAKKYEATLEKCCAEADPSACYGKVLDEFQPLVEEPKNLVKANCELFEKLGEYGFQNALIVRYTQKAPQVSTPTLVEAARNLGKVGSKCCVLPEAQRLPCVEDYISAILNRVCVLHEKTPVSEQVTKCCTGSVVERRPCFSALPVDETYVPKEFKAETFTFHADICSLPEKEKQMKKQAALVELVKHKPKATGPQLRTVLGEFTAFLDKCCKAEDKEACFSEDGPKLVASSQAALA

SEQ ID NO: 7 - protein, 608 aa, Cavia porcellus
MKWVTFISLLFLFSSVYSRGVFRREAHKSEIAHRFNDLGEGHFKGLVLITLSQHLQKSPFEEHVKLVNEVTDFAKACVADESAQNCGKAIATLFGDKVCAIPSLRETYGELADCCAKEDPDRVECFLQHKDDNPNLPPFERPEPEALCTAFKENNDRFIGHYLYEVSRRHPYFYAPELLYYAEKYKNALTECCEAADKAACLTPKLDAIKEKALVSSAQQRLKCASLQKFGERAFKAWSVARLSQKFPKAEFAEISTIVTSLTKVTKECCHGDLLECADDRQELAKYMCEHQDSISSKLKECCVKPTLQKAHCILEIQRDELPTELPDLAVDFVEDKEVCKNFAEAKDVFLGTFLYEYSRRHPEYSIGMLLRIAKGYEAKLEKCCAEADPHACYAKVFDELQPLIDEPKKLVQQNCELFDKLGEYGFQNALAVRYTQKAPQVSTPTLVEYARKLGSVGTKCCSLPETERLSCTENYLALILNRLCILHEKTPVSERVTKCCTESLVNRRPCFSALHVDETYVPKPFHADSFTFHADICTLPEKEKQVKKQMALVELVKHKPKASEEQMKTVMGDFAAFLKKCCDADNKEACFTEDGPKLVAKCQATLA

SEQ ID NO: 8 - protein, 608 aa, Mus musculus
MKWVTFLLLLFVSGSAFSRGVFRREAHKSEIAHRYNDLGEQHFKGLVLIAFSQYLQKCSYDEHAKLVQEVTDFAKTCVADESAANCDKSLHTLFGDKLCAIPNLRENYGELADCCTKQEPERNECFLQHKDDNPSLPPFERPEAEAMCTSFKENPTTFMGHYLHEVARRHPYFYAPELLYYAEQYNEILTQCCAEADKESCLTPKLDGVKEKALVSSVRQRMKCSSMQKFGERAFKAWAVARLSQTFPNADFAEITKLATDLTKVNKECCHGDLLECADDRAELAKYMCENQATISSKLQTCCDKPLLKKAHCLSEVEHDTMPADLPAIAADFVEDQEVCKNYAEAKDVFLGTFLYEYSRRHPDYSVSLLLRLAKKYEATLEKCCAEANPPACYGTVLAEFQPLVEEPKNLVKTNCDLYEKLGEYGFQNAILVRYTQKAPQVSTPTLVEAARNLGRVGTKCCTLPEDQRLPCVEDYLSAILNRVCLLHEKTPVSEHVTKCCSGSLVERRPCFSALTVDETYVPKEFKAETFTFHSDICTLPEKEKQIKKQTALAELVKHKPKATAEQLKTVMDDFAQFLDTCCKAADKDTCFSTEGPNLVTRCKDALA

SEQ ID NO: 9 - protein, 608 aa, Rattus norvegicus
MKWVTFLLLLFISGSAFSRGVFRREAHKSEIAHRFKDLGEQHFKGLVLIAFSQYLQKCPYEEHIKLVQEVTDFAKTCVADENAENCDKSIHTLFGDKLCAIPKLRDNYGELADCCAKQEPERNECFLQHKDDNPNLPPFQRPEAEAMCTSFQENPTSFLGHYLHEVARRHPYFYAPELLYYAEKYNEVLTQCCTESDKAACLTPKLDAVKEKALVAAVRQRMKCSSMQRFGERAFKAWAVARMSQRFPNAEFAEITKLATDVTKINKECCHGDLLECADDRAELAKYMCENQATISSKLQACCDKPVLQKSQCLAEIEHDNIPADLPSIAADFVEDKEVCKNYAEAKDVFLGTFLYEYSRRHPDYSVSLLLRLAKKYEATLEKCCAEGDPPACYGTVLAEFQPLVEEPKNLVKTNCELYEKLGEYGFQNAVLVRYTQKAPQVSTPTLVEAARNLGRVGTKCCTLPEAQRLPCVEDYLSAILNRLCVLHEKTPVSEKVTKCCSGSLVERRPCFSALTVDETYVPKEFKAETFTFHSDICTLPDKEKQIKKQTALAELVKHKPKATEDQLKTVMGDFAQFVDKCCKAADKDNCFATEGPNLVARSKEALA

SEQ ID NO: 10 - protein, 607 aa, Bos taurus
MKWVTFISLLLLFSSAYSRGVFRRDTHKSEIAHRFKDLGEEHFKGLVLIAFSQYLQQCPFDEHVKLVNELTEFAKTCVADESHAGCEKSLHTLFGDELCKVASLRETYGDMADCCEKQEPERNECFLSHKDDSPDLPKLKPDPNTLCDEFKADEKKFWGKYLYEIARRHPYFYAPELLYYANKYNGVFQECCQAEDKGACLLPKIETMREKVLASSARQRLRCASIQKFGERALKAWSVARLSQKFPKAEFVEVTKLVTDLTKVHKECCHGDLLECADDRADLAKYICDNQDTISSKLKECCDKPLLEKSHCIAEVEKDAIPENLPPLTADFAEDKDVCKNYQEAKDAFLGSFLYEYSRRHPEYAVSVLLRLAKEYEATLEECCAKDDPHACYSTVFDKLKHLVDEPQNLIKQNCDQFEKLGEYGFQNALIVRYTRKVPQVSTPTLVEVSRSLGKVGTRCCTKPESERMPCTEDYLSLILNRLCVLHEKTPVSEKVTKCCTESLVNRRPCFSALTPDETYVPKAFDEKLFTFHADICTLPDTEKQIKKQTALVELLKHKPKATEEQLKTVMENFVAFVDKCCAADDKEACFAVEGPKLVVSTQTALA

SEQ ID NO: 11 - protein, 607 aa, Equus caballus
MKWVTFVSLLFLFSSAYSRGVLRRDTHKSEIAHRFNDLGEKHFKGLVLVAFSQYLQQCPFEDHVKLVNEVTEFAKKCAADESAENCDKSLHTLFGDKLCTVATLRATYGELADCCEKQEPERNECFLTHKDDHPNLPKLKPEPDAQCAAFQEDPDKFLGKYLYEVARRHPYFYGPELLFHAEEYKADFTECCPADDKLACLIPKLDALKERILLSSAKERLKCSSFQNFGERAVKAWSVARLSQKFPKADFAEVSKIVTDLTKVHKECCHGDLLECADDRADLAKYICEHQDSISGKLKACCDKPLLQKSHCIAEVKEDDLPSDLPALAADFAEDKEICKHYKDAKDVFLGTFLYEYSRRHPDYSVSLLLRIAKTYEATLEKCCAEADPPACYRTVFDQFTPLVEEPKSLVKKNCDLFEEVGEYDFQNALIVRYTKKAPQVSTPTLVEIGRTLGKVGSRCCKLPESERLPCSENHLALALNRLCVLHEKTPVSEKITKCCTDSLAERRPCFSALELDEGYVPKEFKAETFTFHADICTLPEDEKQIKKQSALAELVKHKPKATKEQLKTVLGNFSAFVAKCCGREDKEACFAEEGPKLVASSQLALA

SEQ ID NO: 12 - protein, 607 aa, Equus asinus
MKWVTFVSLLFLFSSAYFRGVLRRDTHKSEIAHRFNDLGEKHFKGLVLVAFSQYLQQCPFEDHVKLVNEVTEFAKKCAADESAENCDKSLHTLFGDKLCTVATLRATYGELADCCEKQEPERNECFLTHKDDHPNLPKLKPEPDAQCAAFQEDPDKFLGKYLYEVARRHPYFYGPELLFHAEEYKADFTECCPADDKAGCLIPKLDALKERILLSSAKERLKCSSFQKFGERAFKAWSVARLSQKFPKADFAEVSKIVTDLTKVHKECCHGDLLECADDRADLTKYICEHQDSISGKLKACCDKPLLQKSHCIAEVKEDDLPSDLPALAADFAEDKEICKHYKDAKDVFLGTFLYEYSRRHPDYSVSLLLRIAKTYEATLEKCCAEADPPACYATVFDQFTPLVEEPKSLVKKNCDLFEEVGEYDFQNALIVRYTKKAPQVSTPTLVEIGRTLGKVGSRCCKLPESERLPCSENHLALALNRLCVLHEKTPVSEKITKCCTDSLAERRPCFSALELDEGYIPKEFKAETFTFHADICTLPEDEKQIKKQSALAELVKHKPKATKEQLKTVLGNFSAFVAKCCGAEDKEACFAEEGPKLVASSQLALA

SEQ ID NO: 13 - protein, 608 aa, Oryctolagus cuniculus
MKWVTFISLLFLFSSAYSRGVFRREAHKSEIAHRFNDVGEEHFIGLVLITFSQYLQKCPYEEHAKLVKEVTDLAKACVADESAANCDKSLHDIFGDKICALPSLRDTYGDVADCCEKKEPERNECFLHHKDDKPDLPPFARPEADVLCKAFHDDEKAFFGHYLYEVARRHPYFYAPELLYYAQKYKAILTECCEAADKGACLTPKLDALEGKSLISAAQERLRCASIQKFGDRAYKAWALVRLSQRFPKADFTDISKIVTDLTKVHKECCHGDLLECADDRADLAKYMCEHQETISSHLKECCDKPILEKAHCIYGLHNDETPAGLPAVAEEFVEDKDVCKNYEEAKDLFLGKFLYEYSRRHPDYSVVLLLRLGKAYEATLKKCCATDDPHACYAKVLDEFQPLVDEPKNLVKQNCELYEQLGDYNFQNALLVRYTKKVPQVSTPTLVEISRSLGKVGSKCCKHPEAERLPCVEDYLSVVLNRLCVLHEKTPVSEKVTKCCSESLVDRRPCFSALGPDETYVPKEFNAETFTFHADICTLPETERKIKKQTALVELVKHKPHATNDQLKTVVGEFTALLDKCCSAEDKEACFAVEGPKLVESSKATLG

SEQ ID NO: 14 - protein, 583 aa, Capra hircus
DTHKSEIAHRFNDLGEENFQGLVLIAFSQYLQQCPFDEHVKLVKELTEFAKTCVADESHAGCDKSLHTLFGDELCKVATLRETYGDMADCCEKQEPERNECFLKHKDDSPDLPKLKPEPDTLCAEFKADEKKFWGKYLYEVARRHPYFYAPELLYYANKYNGVFQECCQAEDKGACLLPKIETMREKVLASSARQRLRCASIQKFGERALKAWSVARLSQKFPKADFTDVTKIVTDLTKVHKECCHGDLLECADDRADLAKYICDHQDTLSSKLKECCDKPVLEKSHCIAEIDKDAVPENLPPLTADFAEDKEVCKNYQEAKDVFLGSFLYEYSRRHPEYAVSVLLRLAKEYEATLEDCCAKEDPHACYATVFDKLKHLVDEPQNLIKKNCELFEKHGEYGFQNALIVRYTRKAPQVSTPTLVEISRSLGKVGTKCCAKPESERMPCTEDYLSLILNRLCVLHEKTPVSEKVTKCCTESLVNRRPCFSDLTLDETYVPKPFDGESFTFHADICTLPDTEKQIKKQTALVELLKHKPKATDEQLKTVMENFVAFVDKCCAADDKEGCFLLEGPKLVASTQAALA

SEQ ID NO: 15 - protein, 607 aa, Ovis aries
MKWVTFISLLLLFSSAYSRGVFRRDTHKSEIAHRFNDLGEENFQGLVLIAFSQYLQQCPFDEHVKLVKELTEFAKTCVADESHAGCDKSLHTLFGDELCKVATLRETYGDMADCCEKQEPERNECFLNHKDDSPDLPKLKPEPDTLCAEFKADEKKFWGKYLYEVARRHPYFYAPELLYYANKYNGVFQECCQAEDKGACLLPKIDAMREKVLASSARQRLRCASIQKFGERALKAWSVARLSQKFPKADFTDVTKIVTDLTKVHKECCHGDLLECADDRADLAKYICDHQDALSSKLKECCDKPVLEKSHCIAEVDKDAVPENLPPLTADFAEDKEVCKNYQEAKDVFLGSFLYEYSRRHPEYAVSVLLRLAKEYEATLEDCCAKEDPHACYATVFDKLKHLVDEPQNLIKKNCELFEKHGEYGFQNALIVRYTRKAPQVSTPTLVEISRSLGKVGTKCCAKPESERMPCTEDYLSLILNRLCVLHEKTPVSEKVTKCCTESLVNRRPCFSDLTLDETYVPKPFDEKFFTFHADICTLPDTEKQIKKQTALVELLKHKPKATDEQLKTVMENFVAFVDKCCAADDKEGCFVLEGPKLVASTQAALA

SEQ ID NO: 16 - protein, 608 aa, canis lupus familiaris
MKWVTFISLFFLFSSAYSRGLVRREAYKSEIAHRYNDLGEEHFRGLVLVAFSQYLQQCPFEDHVKLAKEVTEFAKACAAEESGANCDKSLHTLFGDKLCTVASLRDKYGDMADCCEKQEPDRNECFLAHKDDNPGFPPLVAPEPDALCAAFQDNEQLFLGKYLYEIARRHPYFYAPELLYYAQQYKGVFAECCQAADKAACLGPKIEALREKVLLSSAKERFKCASLQKFGDRAFKAWSVARLSQRFPKADFAEISKVVTDLTKVHKECCHGDLLECADDRADLAKYMCENQDSISTKLKECCDKPVLEKSQCLAEVERDELPGDLPSLAADFVEDKEVCKNYQEAKDVFLGTFLYEYARRHPEYSVSLLLRLAKEYEATLEKCCATDDPPTCYAKVLDEFKPLVDEPQNLVKTNCELFEKLGEYGFQNALLVRYTKKAPQVSTPTLVEVSRKLGKVGTKCCKKPESERMSCAEDFLSVVLNRLCVLHEKTPVSERVTKCCSESLVNRRPCFSGLEVDETYVPKEFNAETFTFHADLCTLPEAEKQVKKQTALVELLKHKPKATDEQLKTVMGDFGAFVEKCCAAENKEGCFSEEGPKLVAAAQAALV

SEQ ID NO: 17 - protein, 615 aa, Gallus gallus
MKWVTLISFIFLFSSATSRNLQRFARDAEHKSEIAHRYNDLKEETFKAVAMITFAQYLQRCSYEGLSKLVKDVVDLAQKCVANEDAPECSKPLPSIILDEICQVEKLRDSYGAMADCCSKADPERNECFLSFKVSQPDFVQPYQRPASDVICQEYQDNRVSFLGHFIYSVARRHPFLYAPAILSFAVDFEHALQSCCKESDVGACLDTKEIVMREKAKGVSVKQQYFCGILKQFGDRVFQARQLIYLSQKYPKAPFSEVSKFVHDSIGVHKECCEGDMVECMDDMARMMSNLCSQQDVFSGKIKDCCEKPIVERSQCIMEAEFDEKPADLPSLVEKYIEDKEVCKSFEAGHDAFMAEFVYEYSRRHPEFSIQLIMRIAKGYESLLEKCCKTDNPAECYANAQEQLNQHIKETQDVVKTNCDLLHDHGEADFLKSILIRYTKKMPQVPTDLLLETGKKMTTIGTKCCQLGEDRRMACSEGYLSIVIHDTCRKQETTPINDNVSQCCSQLYANRRPCFTAMGVDTKYVPPPFNPDMFSFDEKLCSAPAEEREVGQMKLLINLIKRKPQMTEEQIKTIADGFTAMVDKCCKQSDINTCFGEEGANLIVQSRATLGIGA

SEQ ID NO: 18 - protein, 607 aa, Sus scrofa
MKWVTFISLLFLFSSAYSRGVFRRDTYKSEIAHRFKDLGEQYFKGLVLIAFSQHLQQCPYEEHVKLVREVTEFAKTCVADESAENCDKSIHTLFGDKLCAIPSLREHYGDLADCCEKEEPERNECFLQHKNDNPDIPKLKPDPVALCADFQEDEQKFWGKYLYEIARRHPYFYAPELLYYAIIYKDVFSECCQAADKAACLLPKIEHLREKVLTSAAKQRLKCASIQKFGERAFKAWSLARLSQRFPKADFTEISKIVTDLAKVHKECCHGDLLECADDRADLAKYICENQDTISTKLKECCDKPLLEKSHCIAEAKRDELPADLNPLEHDFVEDKEVCKNYKEAKHVFLGTFLYEYSRRHPDYSVSLLLRIAKIYEATLEDCCAKEDPPACYATVFDKFQPLVDEPKNLIKQNCELFEKLGEYGFQNALIVRYTKKVPQVSTPTLVEVARKLGLVGSRCCKRPEEERLSCAEDYLSLVLNRLCVLHEKTPVSEKVTKCCTESLVNRRPCFSALTPDETYKPKEFVEGTFTFHADLCTLPEDEKQIKKQTALVELLKHKPHATEEQLRTVLGNFAAFVQKCCAAPDHEACFAVEGPKFVIEIRGILA

SEQ ID NO: 19 - protein, 205 aa, Artificial sequence [sequence omitted]

SEQ ID NO: 20 - protein, 403 aa, Artificial sequence
  Artificial albumin variant: human serum albumin domain 2 and human serum albumin domain 3
DELRDEGKASSAKQRLKCASLQKFGERAFKAWAVARLSQRFPKAEFAEVSKLVTDLTKVHTECCHGDLLECADDRADLAKYICENQDSISSKLKECCEKPLLEKSHCIAEVENDEMPADLPSLAADFVESKDVCKNYAEAKDVFLGMFLYEYARRHPDYSVVLLLRLAKTYETTLEKCCAAADPHECYAKVFDEFKPLVEEPQNLIKQNCELFEQLGEYKFQNALLVRYTKKVPQVSTPTLVEVSRNLGKVGSKCCKHPEAKRMPCAEDYLSVVLNQLCVLHEKTPVSDRVTKCCTESLVNRRPCFSALEVDETYVPKEFNAETFTFHADICTLSEKERQIKKQTALVELVKHKPKATKEQLKAVMDDFAAFVEKCCKADDKETCFAEEGKKLVAASQAALGL

SEQ ID NO: 21 - protein, 399 aa, Artificial sequence
  Artificial albumin variant: human serum albumin domain 1 and human serum albumin domain 3
DAHKSEVAHRFKDLGEENFKALVLIAFAQYLQQCPFEDHVKLVNEVTEFAKTCVADESAENCDKSLHTLFGDKLCTVATLRETYGEMADCCAKQEPERNECFLQHKDDNPNLPRLVRPEVDVMCTAFHDNEETFLKKYLYEIARRHPYFYAPELLFFAKRYKAAFTECCQAADKAACLLPKLDELRDEGKASSAVEEPQNLIKQNCELFEQLGEYKFQNALLVRYTKKVPQVSTPTLVEVSRNLGKVGSKCCKHPEAKRMPCAEDYLSVVLNQLCVLHEKTPVSDRVTKCCTESLVNRRPCFSALEVDETYVPKEFNAETFTFHADICTLSEKERQIKKQTALVELVKHKPKATKEQLKAVMDDFAAFVEKCCKADDKETCFAEEGKKLVAASQAALGL

SEQ ID NO: 22 - protein, 410 aa, Artificial sequence
  Artificial albumin variant: two consecutive copies of human serum albumin domain 3
VEEPQNLIKQNCELFEQLGEYKFQNALLVRYTKKVPQVSTPTLVEVSRNLGKVGSKCCKHPEAKRMPCAEDYLSVVLNQLCVLHEKTPVSDRVTKCCTESLVNRRPCFSALEVDETYVPKEFNAETFTFHADICTLSEKERQIKKQTALVELVKHKPKATKEQLKAVMDDFAAFVEKCCKADDKETCFAEEGKKLVAASQAALGLVEEPQNLIKQNCELFEQLGEYKFQNALLVRYTKKVPQVSTPTLVEVSRNLGKVGSKCCKHPEAKRMPCAEDYLSVVLNQLCVLHEKTPVSDRVTKCCTESLVNRRPCFSALEVDETYVPKEFNAETFTFHADICTLSEKERQIKKQTALVELVKHKPKATKEQLKAVMDDFAAFVEKCCKADDKETCFAEEGKKLVAASQAALGL

SEQ ID NO: 23 - protein, 615 aa, Artificial Sequence
  HSA Domain III + HSA Domain III + HSA Domain III
VEEPQNLIKQNCELFEQLGEYKFQNALLVRYTKKVPQVSTPTLVEVSRNLGKVGSKCCKHPEAKRMPCAEDYLSVVLNQLCVLHEKTPVSDRVTKCCTESLVNRRPCFSALEVDETYVPKEFNAETFTFHADICTLSEKERQIKKQTALVELVKHKPKATKEQLKAVMDDFAAFVEKCCKADDKETCFAEEGKKLVAASQAALGLVEEPQNLIKQNCELFEQLGEYKFQNALLVRYTKKVPQVSTPTLVEVSRNLGKVGSKCCKHPEAKRMPCAEDYLSVVLNQLCVLHEKTPVSDRVTKCCTESLVNRRPCFSALEVDETYVPKEFNAETFTFHADICTLSEKERQIKKQTALVELVKHKPKATKEQLKAVMDDFAAFVEKCCKADDKETCFAEEGKKLVAASQAALGLVEEPQNLIKQNCELFEQLGEYKFQNALLVRYTKKVPQVSTPTLVEVSRNLGKVGSKCCKHPEAKRMPCAEDYLSVVLNQLCVLHEKTPVSDRVTKCCTESLVNRRPCFSALEVDETYVPKEFNAETFTFHADICTLSEKERQIKKQTALVELVKHKPKATKEQLKAVMDDFAAFVEKCCKADDKETCFAEEGKKLVAASQAALGL

SEQ ID NO: 24 - protein, 604 aa, Artificial Sequence
  HSA Domain I + HSA Domain III + HSA Domain III
DAHKSEVAHRFKDLGEENFKALVLIAFAQYLQQCPFEDHVKLVNEVTEFAKTCVADESAENCDKSLHTLFGDKLCTVATLRETYGEMADCCAKQEPERNECFLQHKDDNPNLPRLVRPEVDVMCTAFHDNEETFLKKYLYEIARRHPYFYAPELLFFAKRYKAAFTECCQAADKAACLLPKLDELRDEGKASSAVEEPQNLIKQNCELFEQLGEYKFQNALLVRYTKKVPQVSTPTLVEVSRNLGKVGSKCCKHPEAKRMPCAEDYLSVVLNQLCVLHEKTPVSDRVTKCCTESLVNRRPCFSALEVDETYVPKEFNAETFTFHADICTLSEKERQIKKQTALVELVKHKPKATKEQLKAVMDDFAAFVEKCCKADDKETCFAEEGKKLVAASQAALGLVEEPQNLIKQNCELFEQLGEYKFQNALLVRYTKKVPQVSTPTLVEVSRNLGKVGSKCCKHPEAKRMPCAEDYLSVVLNQLCVLHEKTPVSDRVTKCCTESLVNRRPCFSALEVDETYVPKEFNAETFTFHADICTLSEKERQIKKQTALVELVKHKPKATKEQLKAVMDDFAAFVEKCCKADDKETCFAEEGKKLVAASQAALGL

SEQ ID NO: 25 - DNA, 1758 bp, Artificial Sequence
  HSA coding sequence mutated to introduce restriction enzyme sites
gatgcacacaagagtgaggttgctcatcggtttaaagatttgggagaagaaaatttcaaagccttggtgttgattgcctttgctcagtatcttcagcagtgtccatttgaagatcatgtaaaattagtgaatgaagtaactgaatttgcaaaaacatgtgttgctgatgagtccgcggaaaattgtgacaaatcacttcataccctttttggagacaaattatgcacagttgcaactcttcgtgaaacctatggtgaaatggctgactgctgtgcaaaacaagaacctgagagaaatgaatgcttcttgcaacacaaagatgacaacccaaacctcccccgattggtgagaccagaggttgatgtgatgtgcactgcttttcatgacaatgaagagacatttttgaaaaaatacttatatgaaattgccagaagacatccttacttttatgccccggaactccttttctttgctaaaaggtataaagctgcttttacagaatgttgccaagctgctgataaagctgcctgcctgttgccaaagctcgatgaacttcgggatgaagggaaggctagctctgccaaacagagactcaagtgtgccagtctccaaaaatttggagaaagagctttcaaagcatgggcagtagctcgcctgagccagagatttcccaaagctgagtttgcagaagtttccaagttagtgacagatcttaccaaagtccacacggaatgctgccatggagatctgctcgagtgtgctgatgacagggcggaccttgccaagtatatctgtgaaaatcaagattcgatctccagtaaactgaaggaatgctgtgaaaaacctctgttggaaaaatcccactgcattgccgaagtggaaaatgatgagatgcctgctgacttgccttcattagctgctgattttgttgaaagtaaggatgtttgcaaaaactatgctgaggcaaaggatgtcttcctgggcatgtttttgtatgaatatgcaagaaggcatcctgattactctgtcgtgctgctgctgagacttgccaagacatatgaaaccactctagagaagtgctgtgccgctgctgatcctcatgaatgctatgccaaagtgttcgatgaatttaaacctcttgtggaagagcctcagaatttaatcaaacaaaattgtgagctttttgagcagcttggagagtacaaattccagaatgcgctattagttcgttacaccaagaaagtaccccaagtgtcaactccaactcttgtagaggtctcaagaaacctaggaaaagtgggatccaaatgttgtaaacatcctgaagcaaaaagaatgccctgtgcagaagactatctatccgtggtcctgaaccagttatgtgtgttgcatgagaaaacgccagtaagtgacagagtcaccaaatgctgcacagaatccttggtgaacaggcgaccatgcttttcagctctggaagtcgacgaaacatacgttcccaaagagtttaatgctgaaacattcaccttccatgcagatatatgcacactttctgagaaggagagacaaatcaagaaacaaactgcacttgttgagctcgtgaaacacaagcccaaggcaacaaaagagcaactgaaagctgttatggatgatttcgcagcttttgtagagaagtgctgcaaggctgacgataaggagacctgctttgccgaggagggtaaaaaacttgttgctgcaagtcaagctgccttaggcttataa

SEQ ID NO: 26 - protein, 290 aa, Homo sapiens
  misc_feature (1)..(290): Truncated heavy chain of the major histocompatibility complex class I-like Fc receptor (FCGRT) (together, SEQ ID No. 30 and SEQ ID No. 31 form FcRN)
  misc_feature (1)..(290): Truncated heavy chain of the major histocompatibility complex class I-like Fc receptor (FCGRT) (together, SEQ ID No. 26 and SEQ ID No. 27 form FcRN)
MGVPRPQPWALGLLLFLLPGSLGAESHLSLLYHLTAVSSPAPGTPAFWVSGWLGPQQYLSYNSLRGEAEPCGAWVWENQVSWYWEKETTDLRIKEKLFLEAFKALGGKGPYTLQGLLGCELGPDNTSVPTAKFALNGEEFMNFDLKQGTWGGDWPEALAISQRWQQQDKAANKELTFLLFSCPHRLREHLERGRGNLEWKEPPSMRLKARPSSPGFSVLTCSAFSFYPPELQLRFLRNGLAAGTGQGDFGPNSDGSFHASSSLTVKSGDEHHYCCIVQHAGLAQPLRVEL

SEQ ID NO: 27 - protein, 119 aa, Homo sapiens
  misc_feature (1)..(119): Beta-2-microglobulin (together, SEQ ID No. 30 and SEQ ID No. 31 form FcRN)
  misc_feature (1)..(119): Beta-2-microglobulin (together, SEQ ID No. 26 and SEQ ID No. 27 form FcRN)
MSRSVALAVLALLSLSGLEAIQRTPKIQVYSRHPAENGKSNFLNCYVSGFHPSDIEVDLLKNGERIEKVEHSDLSFSKDWSFYLLYYTEFTPTEKDEYACRVNHVTLSQPKIVKWDRDM

SEQ ID NO: 28 - DNA, 1758 bp, Artificial Sequence
  Polynucleotide coding sequence (codon optimised for expression in yeast) for human serum albumin
gacgctcacaagtccgaagtcgctcacagattcaaggacttgggtgaagaaaacttcaaggctttggtcttgatcgctttcgctcaatacttgcaacaatgtccattcgaagatcacgtcaagttggtcaacgaagttaccgaattcgctaagacttgtgttgctgacgaatctgctgaaaactgtgacaagtccttgcacaccttgttcggtgataagttgtgtactgttgctaccttgagagaaacctacggtgaaatggctgactgttgtgctaagcaagaaccagaaagaaacgaatgtttcttgcaacacaaggacgacaacccaaacttgccaagattggttagaccagaagttgacgtcatgtgtactgctttccacgacaacgaagaaaccttcttgaagaagtacttgtacgaaattgctagaagacacccatacttctacgctccagaattgttgttcttcgctaagagatacaaggctgctttcaccgaatgttgtcaagctgctgataaggctgcttgtttgttgccaaagttggatgaattgagagacgaaggtaaggcttcttccgctaagcaaagattgaagtgtgcttccttgcaaaagttcggtgaaagagctttcaaggcttgggctgtcgctagattgtctcaaagattcccaaaggctgaattcgctgaagtttctaagttggttactgacttgactaaggttcacactgaatgttgtcacggtgacttgttggaatgtgctgatgacagagctgacttggctaagtacatctgtgaaaaccaagactctatctcttccaagttgaaggaatgttgtgaaaagccattgttggaaaagtctcactgtattgctgaagttgaaaacgatgaaatgccagctgacttgccatctttggctgctgacttcgttgaatctaaggacgtttgtaagaactacgctgaagctaaggacgtcttcttgggtatgttcttgtacgaatacgctagaagacacccagactactccgttgtcttgttgttgagattggctaagacctacgaaactaccttggaaaagtgttgtgctgctgctgacccacacgaatgttacgctaaggttttcgatgaattcaagccattggtcgaagaaccacaaaacttgatcaagcaaaactgtgaattgttcgaacaattgggtgaatacaagttccaaaacgctttgttggttagatacactaagaaggtcccacaagtctccaccccaactttggttgaagtctctagaaacttgggtaaggtcggttctaagtgttgtaagcacccagaagctaagagaatgccatgtgctgaagattacttgtccgtcgttttgaaccaattgtgtgttttgcacgaaaagaccccagtctctgatagagtcaccaagtgttgtactgaatctttggttaacagaagaccatgtttctctgctttggaagtcgacgaaacttacgttccaaaggaattcaacgctgaaactttcaccttccacgctgatatctgtaccttgtccgaaaaggaaagacaaattaagaagcaaactgctttggttgaattggtcaagcacaagccaaaggctactaaggaacaattgaaggctgtcatggatgatttcgctgctttcgttgaaaagtgttgtaaggctgatgataaggaaacttgtttcgctgaagaaggtaagaagttggtcgctgcttcccaagctgctttgggtttgtaa

SEQ ID NO: 29 - protein, 609 aa, Artificial Sequence
  HSA with fusion leader sequence
  signal (1)..(24)
  mat_peptide (25)..(609)
MKWVSFISLLFLFSSAYSRSLDKRDAHKSEVAHRFKDLGEENFKALVLIAFAQYLQQCPFEDHVKLVNEVTEFAKTCVADESAENCDKSLHTLFGDKLCTVATLRETYGEMADCCAKQEPERNECFLQHKDDNPNLPRLVRPEVDVMCTAFHDNEETFLKKYLYEIARRHPYFYAPELLFFAKRYKAAFTECCQAADKAACLLPKLDELRDEGKASSAKQRLKCASLQKFGERAFKAWAVARLSQRFPKAEFAEVSKLVTDLTKVHTECCHGDLLECADDRADLAKYICENQDSISSKLKECCEKPLLEKSHCIAEVENDEMPADLPSLAADFVESKDVCKNYAEAKDVFLGMFLYEYARRHPDYSVVLLLRLAKTYETTLEKCCAAADPHECYAKVFDEFKPLVEEPQNLIKQNCELFEQLGEYKFQNALLVRYTKKVPQVSTPTLVEVSRNLGKVGSKCCKHPEAKRMPCAEDYLSVVLNQLCVLHEKTPVSDRVTKCCTESLVNRRPCFSALEVDETYVPKEFNAETFTFHADICTLSEKERQIKKQTALVELVKHKPKATKEQLKAVMDDFAAFVEKCCKADDKETCFAEEGKKLVAASQAALGL

SEQ ID NO: 30 - protein, 585 aa, Artificial
  HSA C34A
DAHKSEVAHRFKDLGEENFKALVLIAFAQYLQQAPFEDHVKLVNEVTEFAKTCVADESAENCDKSLHTLFGDKLCTVATLRETYGEMADCCAKQEPERNECFLQHKDDNPNLPRLVRPEVDVMCTAFHDNEETFLKKYLYEIARRHPYFYAPELLFFAKRYKAAFTECCQAADKAACLLPKLDELRDEGKASSAKQRLKCASLQKFGERAFKAWAVARLSQRFPKAEFAEVSKLVTDLTKVHTECCHGDLLECADDRADLAKYICENQDSISSKLKECCEKPLLEKSHCIAEVENDEMPADLPSLAADFVESKDVCKNYAEAKDVFLGMFLYEYARRHPDYSVVLLLRLAKTYETTLEKCCAAADPHECYAKVFDEFKPLVEEPQNLIKQNCELFEQLGEYKFQNALLVRYTKKVPQVSTPTLVEVSRNLGKVGSKCCKHPEAKRMPCAEDYLSVVLNQLCVLHEKTPVSDRVTKCCTESLVNRRPCFSALEVDETYVPKEFNAETFTFHADICTLSEKERQIKKQTALVELVKHKPKATKEQLKAVMDDFAAFVEKCCKADDKETCFAEEGKKLVAASQAALGL

SEQ ID NO: 31 - DNA, 36 bp, Artificial Sequence
  C34A reverse primer
ttgttgcaagtattgagcgaaagcgatcaagaccaa

SEQ ID NO: 32 - DNA, 45 bp, Artificial Sequence
  C34A forward primer
ttcgctcaatacttgcaacaagctccattcgaagatcacgtcaag

SEQ ID NO: 33 - DNA, 50 bp, Artificial Sequence
  L24C forward primer
gaagaaaacttcaaggctttggtctgtatcgctttcgctcaatacttgca

SEQ ID NO: 34 - DNA, 48 bp, Artificial Sequence
  F49C forward primer
agttggtcaacgaagttaccgaatgtgctaagacttgtgttgctgacg

SEQ ID NO: 35 - DNA, 48 bp, Artificial Sequence
  V54C forward primer
gttaccgaattcgctaagacttgttgtgctgacgaatccgcggaaaac

SEQ ID NO: 36 - DNA, 49 bp, Artificial Sequence
  D56C forward primer
gaattcgctaagacttgtgttgcttgtgaatccgcggaaaactgtgaca

SEQ ID NO: 37 - DNA, 48 bp, Artificial Sequence
  L66C forward primer
cgcggaaaactgtgacaagtcctgtcacaccttgttcggtgataagtt

SEQ ID NO: 38 - DNA, 49 bp, Artificial Sequence
  A92C forward primer
cggtgaaatggctgactgttgttgtaagcaagaaccagaaagaaacgaa

SEQ ID NO: 39 - DNA, 50 bp, Artificial Sequence
  K93C forward primer
gtgaaatggctgactgttgtgcttgtcaagaaccagaaagaaacgaatgt

SEQ ID NO: 40 - DNA, 50 bp, Artificial Sequence
  Q94C forward primer
aaatggctgactgttgtgctaagtgtgaaccagaaagaaacgaatgtttc

SEQ ID NO: 41 - DNA, 50 bp, Artificial Sequence
  E97C forward primer
actgttgtgctaagcaagaaccatgtagaaacgaatgtttcttgcaacac

SEQ ID NO: 42 - DNA, 50 bp, Artificial Sequence
  H128C forward primer
ttgacgtcatgtgtactgctttctgtgacaacgaagaaaccttcttgaag

SEQ ID NO: 43 - DNA, 49 bp, Artificial Sequence
  F156C forward primer
acttctacgctccagaattgttgtgtttcgctaagagatacaaggctgc

SEQ ID NO: 44 - DNA, 51 bp, Artificial Sequence
  A226C forward primer
agattgtctcaaagattcccaaagtgtgaattcgctgaagtttctaagttg

SEQ ID NO: 45 - DNA, 50 bp, Artificial Sequence
  A227C forward primer
tgtctcaaagattcccaaaggcttgtttcgctgaagtttctaagttggtt

SEQ ID NO: 46 - DNA, 50 bp, Artificial Sequence
  E230C forward primer
gattcccaaaggctgaattcgcttgtgtttctaagttggttactgacttg

SEQ ID NO: 47 - DNA, 51 bp, Artificial Sequence
  D237C forward primer
gctgaagtttctaagttggttacttgtttgactaaggttcacactgaatgt

SEQ ID NO: 48 - DNA, 50 bp, Artificial Sequence
  K240C forward primer
tctaagttggttactgacttgacttgtgttcacactgaatgttgtcacgg

SEQ ID NO: 49 - DNA, 49 bp, Artificial Sequence
  D259C forward primer
ggaatgtgctgatgacagagcttgtttggctaagtacatctgtgaaaac

SEQ ID NO: 50 - DNA, 49 bp, Artificial Sequence
  K262C forward primer
tgatgacagagctgacttggcttgttacatctgtgaaaaccaagactct

SEQ ID NO: 51 - DNA, 51 bp, Artificial Sequence
  N267C forward primer
gacttggctaagtacatctgtgaatgtcaagactctatctcttccaagttg

SEQ ID NO: 52 - DNA, 51 bp, Artificial Sequence
  Q268C forward primer
ttggctaagtacatctgtgaaaactgtgactctatctcttccaagttgaag

SEQ ID NO: 53 - DNA, 51 bp, Artificial Sequence
  I271C forward primer
tacatctgtgaaaaccaagactcttgttcttccaagttgaaggaatgttgt

SEQ ID NO: 54 - DNA, 50 bp, Artificial Sequence
  L275C forward primer
accaagactctatctcttccaagtgtaaggaatgttgtgaaaagccattg

SEQ ID NO: 55 - DNA, 51 bp, Artificial Sequence
  E277C forward primer
gactctatctcttccaagttgaagtgttgttgtgaaaagccattgttggaa

SEQ ID NO: 56 - DNA, 51 bp, Artificial Sequence
  L284C forward primer
aaggaatgttgtgaaaagccattgtgtgaaaagtctcactgtattgctgaa

SEQ ID NO: 57 - DNA, 50 bp, Artificial Sequence
  E294C forward primer
aagtctcactgtattgctgaagtttgtaacgatgaaatgccagctgactt

SEQ ID NO: 58 - DNA, 50 bp, Artificial Sequence
  E311C forward primer
catctttggctgctgacttcgtttgttctaaggacgtttgtaagaactac

SEQ ID NO: 59 - DNA, 49 bp, Artificial Sequence
  K317C forward primer
ttcgttgaatctaaggacgtttgttgtaactacgctgaagctaaggacg

SEQ ID NO: 60 - DNA, 50 bp, Artificial Sequence
  A322C forward primer
gacgtttgtaagaactacgctgaatgtaaggacgtcttcttgggtatgtt

SEQ ID NO: 61 - DNA, 49 bp, Artificial Sequence
  E333C
gtcttcttgggtatgttcttgtactgttacgctagaagacacccagact

SEQ ID NO: 62 - DNA, 48 bp, Artificial Sequence
  D340C forward primer
cgaatacgctagaagacacccatgttactccgttgtcttgttgttgag

SEQ ID NO: 63 - DNA, 48 bp, Artificial Sequence
  E354C forward primer
tgttgagattggctaagacctactgtactaccctcgagaagtgttgtg

SEQ ID NO: 64 - DNA, 48 bp, Artificial Sequence
  E358C forward primer
ctaagacctacgaaactaccctctgtaagtgttgtgctgctgctgacc

SEQ ID NO: 65 - DNA, 46 bp, Artificial Sequence
  K359C forward primer
gacctacgaaactaccctcgagtgttgttgtgctgctgctgaccca

SEQ ID NO: 66 - DNA, 47 bp, Artificial Sequence
  A362C forward primer
aaactaccctcgagaagtgttgttgtgctgctgacccacacgaatgt

SEQ ID NO: 67 - DNA, 50 bp, Artificial Sequence
  E382C forward primer
tcgatgaattcaagccattggtctgtgaaccacaaaacttgatcaagcaa

SEQ ID NO: 68 - DNA, 51 bp, Artificial Sequence
  L398C forward primer
gcaaaactgtgaattgttcgaacaatgtggtgaatacaagttccaaaacgc

SEQ ID NO: 69 - DNA, 35 bp, Artificial Sequence
  L24C reverse primer
gaccaaagccttgaagttttcttcacccaagtcct

SEQ ID NO: 70 - DNA, 35 bp, Artificial Sequence
  F49C reverse primer
ttcggtaacttcgttgaccaacttgacgtgatctt

SEQ ID NO: 71 - DNA, 36 bp, Artificial Sequence
  V54C reverse primer
acaagtcttagcgaattcggtaacttcgttgaccaa

SEQ ID NO: 72 - DNA, 36 bp, Artificial Sequence
  D56C reverse primer
agcaacacaagtcttagcgaattcggtaacttcgtt

SEQ ID NO: 73 - DNA, 33 bp, Artificial Sequence
  L66C reverse primer
ggacttgtcacagttttccgcggattcgtcagc

SEQ ID NO: 74 - DNA, 34 bp, Artificial Sequence
  A92C reverse primer
acaacagtcagccatttcaccgtaggtttctctc

SEQ ID NO: 75 - DNA, 35 bp, Artificial Sequence
  K93C reverse primer
agcacaacagtcagccatttcaccgtaggtttctc

SEQ ID NO: 76 - DNA, 34 bp, Artificial Sequence
  Q94C reverse primer
cttagcacaacagtcagccatttcaccgtaggtt

SEQ ID NO: 77 - DNA, 35 bp, Artificial Sequence
  E97C reverse primer
tggttcttgcttagcacaacagtcagccatttcac

SEQ ID NO: 78 - DNA, 35 bp, Artificial Sequence
  H128C reverse primer
gaaagcagtacacatgacgtcaacttctggtctaa

SEQ ID NO: 79 - DNA, 35 bp, Artificial Sequence
  F156C reverse primer
caacaattctggagcgtagaagtatgggtgtcttc

SEQ ID NO: 80 - DNA, 34 bp, Artificial Sequence
  A226C reverse primer
ctttgggaatctttgagacaatctagcgacagcc

SEQ ID NO: 81 - DNA, 35 bp, Artificial Sequence
  E227C reverse primer
agcctttgggaatctttgagacaatctagcgacag

SEQ ID NO: 82 - DNA, 36 bp, Artificial Sequence
  E230C reverse primer
agcgaattcagcctttgggaatctttgagacaatct

SEQ ID NO: 83 - DNA, 36 bp, Artificial Sequence
  E237C reverse primer
agtaaccaacttagaaacttcagcgaattcagcctt

SEQ ID NO: 84 - DNA, 36 bp, Artificial Sequence
  K240C reverse primer
agtcaagtcagtaaccaacttagaaacttcagcgaa

SEQ ID NO: 85 - DNA, 34 bp, Artificial Sequence
  D259C reverse primer
agctctgtcatcagcacattccaacaagtcaccg

SEQ ID NO: 86 - DNA, 34 bp, Artificial Sequence
  K262C reverse primer
agccaagtcagctctgtcatcagcacattccaac

SEQ ID NO: 87 - DNA, 36 bp, Artificial Sequence
  N267C reverse primer
ttcacagatgtacttagccaagtcagctctgtcatc

SEQ ID NO: 88 - DNA, 35 bp, Artificial Sequence
  Q268C reverse primer
gttttcacagatgtacttagccaagtcagctctgt

SEQ ID NO: 89 - DNA, 36 bp, Artificial Sequence
  I271C reverse primer
agagtcttggttttcacagatgtacttagccaagtc

SEQ ID NO: 90 - DNA, 36 bp, Artificial Sequence
  L275C reverse primer
cttggaagagatagagtcttggttttcacagatgta

SEQ ID NO: 91 - DNA, 37 bp, Artificial Sequence
  E277C reverse primer
cttcaacttggaagagatagagtcttggttttcacag

SEQ ID NO: 92 - DNA, 36 bp, Artificial Sequence
  E284C reverse primer
caatggcttttcacaacattccttcaacttggaaga

SEQ ID NO: 93 - DNA, 36 bp, Artificial Sequence
  E294C reverse primer
aacttcagcaatacagtgagacttttccaacaatgg

SEQ ID NO: 94 - DNA, 34 bp, Artificial Sequence
  E311C reverse primer
aacgaagtcagcagccaaagatggcaagtcagct

SEQ ID NO: 95 - DNA, 34 bp, Artificial Sequence
  K317C reverse primer
acaaacgtccttagattcaacgaagtcagcagcc

SEQ ID NO: 96 - DNA, 37 bp, Artificial Sequence
  A322C reverse primer
ttcagcgtagttcttacaaacgtccttagattcaacg

SEQ ID NO: 97 - DNA, 36 bp, Artificial Sequence
  E333C reverse primer
gtacaagaacatacccaagaagacgtccttagcttc

SEQ ID NO: 98 - DNA, 35 bp, Artificial Sequence
  D340C reverse primer
tgggtgtcttctagcgtattcgtacaagaacatac

SEQ ID NO: 99 - DNA, 35 bp, Artificial Sequence
  E354C reverse primer
gtaggtcttagccaatctcaacaacaagacaacgg

SEQ ID NO: 100 - DNA, 35 bp, Artificial Sequence
  E358C reverse primer
gagggtagtttcgtaggtcttagccaatctcaaca

SEQ ID NO: 101 - DNA, 34 bp, Artificial Sequence
  K359C reverse primer
ctcgagggtagtttcgtaggtcttagccaatctc

SEQ ID NO: 102 - DNA, 35 bp, Artificial Sequence
  A362C reverse primer
acaacacttctcgagggtagtttcgtaggtcttag

SEQ ID NO: 103 - DNA, 35 bp, Artificial Sequence
  E382C reverse primer
gaccaatggcttgaattcatcgaaaaccttagcgt

SEQ ID NO: 104 - DNA, 39 bp, Artificial Sequence
  L398C reverse primer
ttgttcgaacaattcacagttttgcttgatcaagttttg

SEQ ID NO: 105 - protein, 585 aa, Artificial Sequence
  HSA C34A_L24C
DAHKSEVAHRFKDLGEENFKALVCIAFAQYLQQAPFEDHVKLVNEVTEFAKTCVADESAENCDKSLHTLFGDKLCTVATLRETYGEMADCCAKQEPERNECFLQHKDDNPNLPRLVRPEVDVMCTAFHDNEETFLKKYLYEIARRHPYFYAPELLFFAKRYKAAFTECCQAADKAACLLPKLDELRDEGKASSAKQRLKCASLQKFGERAFKAWAVARLSQRFPKAEFAEVSKLVTDLTKVHTECCHGDLLECADDRADLAKYICENQDSISSKLKECCEKPLLEKSHCIAEVENDEMPADLPSLAADFVESKDVCKNYAEAKDVFLGMFLYEYARRHPDYSVVLLLRLAKTYETTLEKCCAAADPHECYAKVFDEFKPLVEEPQNLIKQNCELFEQLGEYKFQNALLVRYTKKVPQVSTPTLVEVSRNLGKVGSKCCKHPEAKRMPCAEDYLSVVLNQLCVLHEKTPVSDRVTKCCTESLVNRRPCFSALEVDETYVPKEFNAETFTFHADICTLSEKERQIKKQTALVELVKHKPKATKEQLKAVMDDFAAFVEKCCKADDKETCFAEEGKKLVAASQAALGL

SEQ ID NO: 106 - protein, 585 aa, Artificial Sequence
  HSA C34A_F49C
DAHKSEVAHRFKDLGEENFKALVLIAFAQYLQQAPFEDHVKLVNEVTECAKTCVADESAENCDKSLHTLFGDKLCTVATLRETYGEMADCCAKQEPERNECFLQHKDDNPNLPRLVRPEVDVMCTAFHDNEETFLKKYLYEIARRHPYFYAPELLFFAKRYKAAFTECCQAADKAACLLPKLDELRDEGKASSAKQRLKCASLQKFGERAFKAWAVARLSQRFPKAEFAEVSKLVTDLTKVHTECCHGDLLECADDRADLAKYICENQDSISSKLKECCEKPLLEKSHCIAEVENDEMPADLPSLAADFVESKDVCKNYAEAKDVFLGMFLYEYARRHPDYSVVLLLRLAKTYETTLEKCCAAADPHECYAKVFDEFKPLVEEPQNLIKQNCELFEQLGEYKFQNALLVRYTKKVPQVSTPTLVEVSRNLGKVGSKCCKHPEAKRMPCAEDYLSVVLNQLCVLHEKTPVSDRVTKCCTESLVNRRPCFSALEVDETYVPKEFNAETFTFHADICTLSEKERQIKKQTALVELVKHKPKATKEQLKAVMDDFAAFVEKCCKADDKETCFAEEGKKLVAASQAALGL

SEQ ID NO: 107 - protein, 585 aa, Artificial Sequence
  HSA C34A_V54C
DAHKSEVAHRFKDLGEENFKALVLIAFAQYLQQAPFEDHVKLVNEVTEFAKTCCADESAENCDKSLHTLFGDKLCTVATLRETYGEMADCCAKQEPERNECFLQHKDDNPNLPRLVRPEVDVMCTAFHDNEETFLKKYLYEIARRHPYFYAPELLFFAKRYKAAFTECCQAADKAACLLPKLDELRDEGKASSAKQRLKCASLQKFGERAFKAWAVARLSQRFPKAEFAEVSKLVTDLTKVHTECCHGDLLECADDRADLAKYICENQDSISSKLKECCEKPLLEKSHCIAEVENDEMPADLPSLAADFVESKDVCKNYAEAKDVFLGMFLYEYARRHPDYSVVLLLRLAKTYETTLEKCCAAADPHECYAKVFDEFKPLVEEPQNLIKQNCELFEQLGEYKFQNALLVRYTKKVPQVSTPTLVEVSRNLGKVGSKCCKHPEAKRMPCAEDYLSVVLNQLCVLHEKTPVSDRVTKCCTESLVNRRPCFSALEVDETYVPKEFNAETFTFHADICTLSEKERQIKKQTALVELVKHKPKATKEQLKAVMDDFAAFVEKCCKADDKETCFAEEGKKLVAASQAALGL

SEQ ID NO: 108 - protein, 585 aa, Artificial Sequence
  HSA C34A_D56C
DAHKSEVAHRFKDLGEENFKALVLIAFAQYLQQAPFEDHVKLVNEVTEFAKTCVACESAENCDKSLHTLFGDKLCTVATLRETYGEMADCCAKQEPERNECFLQHKDDNPNLPRLVRPEVDVMCTAFHDNEETFLKKYLYEIARRHPYFYAPELLFFAKRYKAAFTECCQAADKAACLLPKLDELRDEGKASSAKQRLKCASLQKFGERAFKAWAVARLSQRFPKAEFAEVSKLVTDLTKVHTECCHGDLLECADDRADLAKYICENQDSISSKLKECCEKPLLEKSHCIAEVENDEMPADLPSLAADFVESKDVCKNYAEAKDVFLGMFLYEYARRHPDYSVVLLLRLAKTYETTLEKCCAAADPHECYAKVFDEFKPLVEEPQNLIKQNCELFEQLGEYKFQNALLVRYTKKVPQVSTPTLVEVSRNLGKVGSKCCKHPEAKRMPCAEDYLSVVLNQLCVLHEKTPVSDRVTKCCTESLVNRRPCFSALEVDETYVPKEFNAETFTFHADICTLSEKERQIKKQTALVELVKHKPKATKEQLKAVMDDFAAFVEKCCKADDKETCFAEEGKKLVAASQAALGL

SEQ ID NO: 109 - protein, 585 aa, Artificial Sequence
  HSA C34A_L66C
DAHKSEVAHRFKDLGEENFKALVLIAFAQYLQQAPFEDHVKLVNEVTEFAKTCVADESAENCDKSCHTLFGDKLCTVATLRETYGEMADCCAKQEPERNECFLQHKDDNPNLPRLVRPEVDVMCTAFHDNEETFLKKYLYEIARRHPYFYAPELLFFAKRYKAAFTECCQAADKAACLLPKLDELRDEGKASSAKQRLKCASLQKFGERAFKAWAVARLSQRFPKAEFAEVSKLVTDLTKVHTECCHGDLLECADDRADLAKYICENQDSISSKLKECCEKPLLEKSHCIAEVENDEMPADLPSLAADFVESKDVCKNYAEAKDVFLGMFLYEYARRHPDYSVVLLLRLAKTYETTLEKCCAAADPHECYAKVFDEFKPLVEEPQNLIKQNCELFEQLGEYKFQNALLVRYTKKVPQVSTPTLVEVSRNLGKVGSKCCKHPEAKRMPCAEDYLSVVLNQLCVLHEKTPVSDRVTKCCTESLVNRRPCFSALEVDETYVPKEFNAETFTFHADICTLSEKERQIKKQTALVELVKHKPKATKEQLKAVMDDFAAFVEKCCKADDKETCFAEEGKKLVAASQAALGL

SEQ ID NO: 110 - protein, 585 aa, Artificial Sequence
  HSA C34A_A92C
DAHKSEVAHRFKDLGEENFKALVLIAFAQYLQQAPFEDHVKLVNEVTEFAKTCVADESAENCDKSLHTLFGDKLCTVATLRETYGEMADCCCKQEPERNECFLQHKDDNPNLPRLVRPEVDVMCTAFHDNEETFLKKYLYEIARRHPYFYAPELLFFAKRYKAAFTECCQAADKAACLLPKLDELRDEGKASSAKQRLKCASLQKFGERAFKAWAVARLSQRFPKAEFAEVSKLVTDLTKVHTECCHGDLLECADDRADLAKYICENQDSISSKLKECCEKPLLEKSHCIAEVENDEMPADLPSLAADFVESKDVCKNYAEAKDVFLGMFLYEYARRHPDYSVVLLLRLAKTYETTLEKCCAAADPHECYAKVFDEFKPLVEEPQNLIKQNCELFEQLGEYKFQNALLVRYTKKVPQVSTPTLVEVSRNLGKVGSKCCKHPEAKRMPCAEDYLSVVLNQLCVLHEKTPVSDRVTKCCTESLVNRRPCFSALEVDETYVPKEFNAETFTFHADICTLSEKERQIKKQTALVELVKHKPKATKEQLKAVMDDFAAFVEKCCKADDKETCFAEEGKKLVAASQAALGL

SEQ ID NO: 111 - protein, 585 aa, Artificial Sequence
  HSA C34A_K93C
DAHKSEVAHRFKDLGEENFKALVLIAFAQYLQQAPFEDHVKLVNEVTEFAKTCVADESAENCDKSLHTLFGDKLCTVATLRETYGEMADCCACQEPERNECFLQHKDDNPNLPRLVRPEVDVMCTAFHDNEETFLKKYLYEIARRHPYFYAPELLFFAKRYKAAFTECCQAADKAACLLPKLDELRDEGKASSAKQRLKCASLQKFGERAFKAWAVARLSQRFPKAEFAEVSKLVTDLTKVHTECCHGDLLECADDRADLAKYICENQDSISSKLKECCEKPLLEKSHCIAEVENDEMPADLPSLAADFVESKDVCKNYAEAKDVFLGMFLYEYARRHPDYSVVLLLRLAKTYETTLEKCCAAADPHECYAKVFDEFKPLVEEPQNLIKQNCELFEQLGEYKFQNALLVRYTKKVPQVSTPTLVEVSRNLGKVGSKCCKHPEAKRMPCAEDYLSVVLNQLCVLHEKTPVSDRVTKCCTESLVNRRPCFSALEVDETYVPKEFNAETFTFHADICTLSEKERQIKKQTALVELVKHKPKATKEQLKAVMDDFAAFVEKCCKADDKETCFAEEGKKLVAASQAALGL

SEQ ID NO: 112 - protein, 585 aa, Artificial Sequence
  HSA C34A_Q94C
DAHKSEVAHRFKDLGEENFKALVLIAFAQYLQQAPFEDHVKLVNEVTEFAKTCVADESAENCDKSLHTLFGDKLCTVATLRETYGEMADCCAKCEPERNECFLQHKDDNPNLPRLVRPEVDVMCTAFHDNEETFLKKYLYEIARRHPYFYAPELLFFAKRYKAAFTECCQAADKAACLLPKLDELRDEGKASSAKQRLKCASLQKFGERAFKAWAVARLSQRFPKAEFAEVSKLVTDLTKVHTECCHGDLLECADDRADLAKYICENQDSISSKLKECCEKPLLEKSHCIAEVENDEMPADLPSLAADFVESKDVCKNYAEAKDVFLGMFLYEYARRHPDYSVVLLLRLAKTYETTLEKCCAAADPHECYAKVFDEFKPLVEEPQNLIKQNCELFEQLGEYKFQNALLVRYTKKVPQVSTPTLVEVSRNLGKVGSKCCKHPEAKRMPCAEDYLSVVLNQLCVLHEKTPVSDRVTKCCTESLVNRRPCFSALEVDETYVPKEFNAETFTFHADICTLSEKERQIKKQTALVELVKHKPKATKEQLKAVMDDFAAFVEKCCKADDKETCFAEEGKKLVAASQAALGL

SEQ ID NO: 113 - protein, 585 aa, Artificial Sequence
  HSA C34A_E97C
DAHKSEVAHRFKDLGEENFKALVLIAFAQYLQQAPFEDHVKLVNEVTEFAKTCVADESAENCDKSLHTLFGDKLCTVATLRETYGEMADCCAKQEPCRNECFLQHKDDNPNLPRLVRPEVDVMCTAFHDNEETFLKKYLYEIARRHPYFYAPELLFFAKRYKAAFTECCQAADKAACLLPKLDELRDEGKASSAKQRLKCASLQKFGERAFKAWAVARLSQRFPKAEFAEVSKLVTDLTKVHTECCHGDLLECADDRADLAKYICENQDSISSKLKECCEKPLLEKSHCIAEVENDEMPADLPSLAADFVESKDVCKNYAEAKDVFLGMFLYEYARRHPDYSVVLLLRLAKTYETTLEKCCAAADPHECYAKVFDEFKPLVEEPQNLIKQNCELFEQLGEYKFQNALLVRYTKKVPQVSTPTLVEVSRNLGKVGSKCCKHPEAKRMPCAEDYLSVVLNQLCVLHEKTPVSDRVTKCCTESLVNRRPCFSALEVDETYVPKEFNAETFTFHADICTLSEKERQIKKQTALVELVKHKPKATKEQLKAVMDDFAAFVEKCCKADDKETCFAEEGKKLVAASQAALGL

SEQ ID NO: 114 - protein, 585 aa, Artificial Sequence
  HSA C34A_H128C
DAHKSEVAHRFKDLGEENFKALVLIAFAQYLQQAPFEDHVKLVNEVTEFAKTCVADESAENCDKSLHTLFGDKLCTVATLRETYGEMADCCAKQEPERNECFLQHKDDNPNLPRLVRPEVDVMCTAFCDNEETFLKKYLYEIARRHPYFYAPELLFFAKRYKAAFTECCQAADKAACLLPKLDELRDEGKASSAKQRLKCASLQKFGERAFKAWAVARLSQRFPKAEFAEVSKLVTDLTKVHTECCHGDLLECADDRADLAKYICENQDSISSKLKECCEKPLLEKSHCIAEVENDEMPADLPSLAADFVESKDVCKNYAEAKDVFLGMFLYEYARRHPDYSVVLLLRLAKTYETTLEKCCAAADPHECYAKVFDEFKPLVEEPQNLIKQNCELFEQLGEYKFQNALLVRYTKKVPQVSTPTLVEVSRNLGKVGSKCCKHPEAKRMPCAEDYLSVVLNQLCVLHEKTPVSDRVTKCCTESLVNRRPCFSALEVDETYVPKEFNAETFTFHADICTLSEKERQIKKQTALVELVKHKPKATKEQLKAVMDDFAAFVEKCCKADDKETCFAEEGKKLVAASQAALGL

SEQ ID NO: 115 - protein, 585 aa, Artificial Sequence
  HSA C34A_F156C
DAHKSEVAHRFKDLGEENFKALVLIAFAQYLQQAPFEDHVKLVNEVTEFAKTCVADESAENCDKSLHTLFGDKLCTVATLRETYGEMADCCAKQEPERNECFLQHKDDNPNLPRLVRPEVDVMCTAFHDNEETFLKKYLYEIARRHPYFYAPELLCFAKRYKAAFTECCQAADKAACLLPKLDELRDEGKASSAKQRLKCASLQKFGERAFKAWAVARLSQRFPKAEFAEVSKLVTDLTKVHTECCHGDLLECADDRADLAKYICENQDSISSKLKECCEKPLLEKSHCIAEVENDEMPADLPSLAADFVESKDVCKNYAEAKDVFLGMFLYEYARRHPDYSVVLLLRLAKTYETTLEKCCAAADPHECYAKVFDEFKPLVEEPQNLIKQNCELFEQLGEYKFQNALLVRYTKKVPQVSTPTLVEVSRNLGKVGSKCCKHPEAKRMPCAEDYLSVVLNQLCVLHEKTPVSDRVTKCCTESLVNRRPCFSALEVDETYVPKEFNAETFTFHADICTLSEKERQIKKQTALVELVKHKPKATKEQLKAVMDDFAAFVEKCCKADDKETCFAEEGKKLVAASQAALGL

SEQ ID NO: 116 - protein, 585 aa, Artificial Sequence
  HSA C34A_A226C
DAHKSEVAHRFKDLGEENFKALVLIAFAQYLQQAPFEDHVKLVNEVTEFAKTCVADESAENCDKSLHTLFGDKLCTVATLRETYGEMADCCAKQEPERNECFLQHKDDNPNLPRLVRPEVDVMCTAFHDNEETFLKKYLYEIARRHPYFYAPELLFFAKRYKAAFTECCQAADKAACLLPKLDELRDEGKASSAKQRLKCASLQKFGERAFKAWAVARLSQRFPKCEFAEVSKLVTDLTKVHTECCHGDLLECADDRADLAKYICENQDSISSKLKECCEKPLLEKSHCIAEVENDEMPADLPSLAADFVESKDVCKNYAEAKDVFLGMFLYEYARRHPDYSVVLLLRLAKTYETTLEKCCAAADPHECYAKVFDEFKPLVEEPQNLIKQNCELFEQLGEYKFQNALLVRYTKKVPQVSTPTLVEVSRNLGKVGSKCCKHPEAKRMPCAEDYLSVVLNQLCVLHEKTPVSDRVTKCCTESLVNRRPCFSALEVDETYVPKEFNAETFTFHADICTLSEKERQIKKQTALVELVKHKPKATKEQLKAVMDDFAAFVEKCCKADDKETCFAEEGKKLVAASQAALGL

SEQ ID NO: 117 - protein, 585 aa, Artificial Sequence
  HSA C34A_E227C
DAHKSEVAHRFKDLGEENFKALVLIAFAQYLQQAPFEDHVKLVNEVTEFAKTCVADESAENCDKSLHTLFGDKLCTVATLRETYGEMADCCAKQEPERNECFLQHKDDNPNLPRLVRPEVDVMCTAFHDNEETFLKKYLYEIARRHPYFYAPELLFFAKRYKAAFTECCQAADKAACLLPKLDELRDEGKASSAKQRLKCASLQKFGERAFKAWAVARLSQRFPKACFAEVSKLVTDLTKVHTECCHGDLLECADDRADLAKYICENQDSISSKLKECCEKPLLEKSHCIAEVENDEMPADLPSLAADFVESKDVCKNYAEAKDVFLGMFLYEYARRHPDYSVVLLLRLAKTYETTLEKCCAAADPHECYAKVFDEFKPLVEEPQNLIKQNCELFEQLGEYKFQNALLVRYTKKVPQVSTPTLVEVSRNLGKVGSKCCKHPEAKRMPCAEDYLSVVLNQLCVLHEKTPVSDRVTKCCTESLVNRRPCFSALEVDETYVPKEFNAETFTFHADICTLSEKERQIKKQTALVELVKHKPKATKEQLKAVMDDFAAFVEKCCKADDKETCFAEEGKKLVAASQAALGL

SEQ ID NO: 118 - protein, 585 aa, Artificial Sequence
  HSA C34A_E230C
DAHKSEVAHRFKDLGEENFKALVLIAFAQYLQQAPFEDHVKLVNEVTEFAKTCVADESAENCDKSLHTLFGDKLCTVATLRETYGEMADCCAKQEPERNECFLQHKDDNPNLPRLVRPEVDVMCTAFHDNEETFLKKYLYEIARRHPYFYAPELLFFAKRYKAAFTECCQAADKAACLLPKLDELRDEGKASSAKQRLKCASLQKFGERAFKAWAVARLSQRFPKAEFACVSKLVTDLTKVHTECCHGDLLECADDRADLAKYICENQDSISSKLKECCEKPLLEKSHCIAEVENDEMPADLPSLAADFVESKDVCKNYAEAKDVFLGMFLYEYARRHPDYSVVLLLRLAKTYETTLEKCCAAADPHECYAKVFDEFKPLVEEPQNLIKQNCELFEQLGEYKFQNALLVRYTKKVPQVSTPTLVEVSRNLGKVGSKCCKHPEAKRMPCAEDYLSVVLNQLCVLHEKTPVSDRVTKCCTESLVNRRPCFSALEVDETYVPKEFNAETFTFHADICTLSEKERQIKKQTALVELVKHKPKATKEQLKAVMDDFAAFVEKCCKADDKETCFAEEGKKLVAASQAALGL

SEQ ID NO: 119 - protein, 585 aa, Artificial Sequence
  HSA C34A_D237C
DAHKSEVAHRFKDLGEENFKALVLIAFAQYLQQAPFEDHVKLVNEVTEFAKTCVADESAENCDKSLHTLFGDKLCTVATLRETYGEMADCCAKQEPERNECFLQHKDDNPNLPRLVRPEVDVMCTAFHDNEETFLKKYLYEIARRHPYFYAPELLFFAKRYKAAFTECCQAADKAACLLPKLDELRDEGKASSAKQRLKCASLQKFGERAFKAWAVARLSQRFPKAEFAEVSKLVTCLTKVHTECCHGDLLECADDRADLAKYICENQDSISSKLKECCEKPLLEKSHCIAEVENDEMPADLPSLAADFVESKDVCKNYAEAKDVFLGMFLYEYARRHPDYSVVLLLRLAKTYETTLEKCCAAADPHECYAKVFDEFKPLVEEPQNLIKQNCELFEQLGEYKFQNALLVRYTKKVPQVSTPTLVEVSRNLGKVGSKCCKHPEAKRMPCAEDYLSVVLNQLCVLHEKTPVSDRVTKCCTESLVNRRPCFSALEVDETYVPKEFNAETFTFHADICTLSEKERQIKKQTALVELVKHKPKATKEQLKAVMDDFAAFVEKCCKADDKETCFAEEGKKLVAASQAALGL

SEQ ID NO: 120 - protein, 585 aa, Artificial Sequence
  HSA C34A_K240C
DAHKSEVAHRFKDLGEENFKALVLIAFAQYLQQAPFEDHVKLVNEVTEFAKTCVADESAENCDKSLHTLFGDKLCTVATLRETYGEMADCCAKQEPERNECFLQHKDDNPNLPRLVRPEVDVMCTAFHDNEETFLKKYLYEIARRHPYFYAPELLFFAKRYKAAFTECCQAADKAACLLPKLDELRDEGKASSAKQRLKCASLQKFGERAFKAWAVARLSQRFPKAEFAEVSKLVTDLTCVHTECCHGDLLECADDRADLAKYICENQDSISSKLKECCEKPLLEKSHCIAEVENDEMPADLPSLAADFVESKDVCKNYAEAKDVFLGMFLYEYARRHPDYSVVLLLRLAKTYETTLEKCCAAADPHECYAKVFDEFKPLVEEPQNLIKQNCELFEQLGEYKFQNALLVRYTKKVPQVSTPTLVEVSRNLGKVGSKCCKHPEAKRMPCAEDYLSVVLNQLCVLHEKTPVSDRVTKCCTESLVNRRPCFSALEVDETYVPKEFNAETFTFHADICTLSEKERQIKKQTALVELVKHKPKATKEQLKAVMDDFAAFVEKCCKADDKETCFAEEGKKLVAASQAALGL

SEQ ID NO: 121 - protein, 585 aa, Artificial Sequence
  HSA C34A_D259C
DAHKSEVAHRFKDLGEENFKALVLIAFAQYLQQAPFEDHVKLVNEVTEFAKTCVADESAENCDKSLHTLFGDKLCTVATLRETYGEMADCCAKQEPERNECFLQHKDDNPNLPRLVRPEVDVMCTAFHDNEETFLKKYLYEIARRHPYFYAPELLFFAKRYKAAFTECCQAADKAACLLPKLDELRDEGKASSAKQRLKCASLQKFGERAFKAWAVARLSQRFPKAEFAEVSKLVTDLTKVHTECCHGDLLECADDRACLAKYICENQDSISSKLKECCEKPLLEKSHCIAEVENDEMPADLPSLAADFVESKDVCKNYAEAKDVFLGMFLYEYARRHPDYSVVLLLRLAKTYETTLEKCCAAADPHECYAKVFDEFKPLVEEPQNLIKQNCELFEQLGEYKFQNALLVRYTKKVPQVSTPTLVEVSRNLGKVGSKCCKHPEAKRMPCAEDYLSVVLNQLCVLHEKTPVSDRVTKCCTESLVNRRPCFSALEVDETYVPKEFNAETFTFHADICTLSEKERQIKKQTALVELVKHKPKATKEQLKAVMDDFAAFVEKCCKADDKETCFAEEGKKLVAASQAALGL

SEQ ID NO: 122 - protein, 585 aa, Artificial Sequence
  HSA C34A_K262C
DAHKSEVAHRFKDLGEENFKALVLIAFAQYLQQAPFEDHVKLVNEVTEFAKTCVADESAENCDKSLHTLFGDKLCTVATLRETYGEMADCCAKQEPERNECFLQHKDDNPNLPRLVRPEVDVMCTAFHDNEETFLKKYLYEIARRHPYFYAPELLFFAKRYKAAFTECCQAADKAACLLPKLDELRDEGKASSAKQRLKCASLQKFGERAFKAWAVARLSQRFPKAEFAEVSKLVTDLTKVHTECCHGDLLECADDRADLACYICENQDSISSKLKECCEKPLLEKSHCIAEVENDEMPADLPSLAADFVESKDVCKNYAEAKDVFLGMFLYEYARRHPDYSVVLLLRLAKTYETTLEKCCAAADPHECYAKVFDEFKPLVEEPQNLIKQNCELFEQLGEYKFQNALLVRYTKKVPQVSTPTLVEVSRNLGKVGSKCCKHPEAKRMPCAEDYLSVVLNQLCVLHEKTPVSDRVTKCCTESLVNRRPCFSALEVDETYVPKEFNAETFTFHADICTLSEKERQIKKQTALVELVKHKPKATKEQLKAVMDDFAAFVEKCCKADDKETCFAEEGKKLVAASQAALGL

SEQ ID NO: 123 - protein, 585 aa, Artificial Sequence
  HSA C34A_N267C
DAHKSEVAHRFKDLGEENFKALVLIAFAQYLQQAPFEDHVKLVNEVTEFAKTCVADESAENCDKSLHTLFGDKLCTVATLRETYGEMADCCAKQEPERNECFLQHKDDNPNLPRLVRPEVDVMCTAFHDNEETFLKKYLYEIARRHPYFYAPELLFFAKRYKAAFTECCQAADKAACLLPKLDELRDEGKASSAKQRLKCASLQKFGERAFKAWAVARLSQRFPKAEFAEVSKLVTDLTKVHTECCHGDLLECADDRADLAKYICECQDSISSKLKECCEKPLLEKSHCIAEVENDEMPADLPSLAADFVESKDVCKNYAEAKDVFLGMFLYEYARRHPDYSVVLLLRLAKTYETTLEKCCAAADPHECYAKVFDEFKPLVEEPQNLIKQNCELFEQLGEYKFQNALLVRYTKKVPQVSTPTLVEVSRNLGKVGSKCCKHPEAKRMPCAEDYLSVVLNQLCVLHEKTPVSDRVTKCCTESLVNRRPCFSALEVDETYVPKEFNAETFTFHADICTLSEKERQIKKQTALVELVKHKPKATKEQLKAVMDDFAAFVEKCCKADDKETCFAEEGKKLVAASQAALGL

SEQ ID NO: 124 - protein, 585 aa, Artificial Sequence
  HSA C34A_Q268C
DAHKSEVAHRFKDLGEENFKALVLIAFAQYLQQAPFEDHVKLVNEVTEFAKTCVADESAENCDKSLHTLFGDKLCTVATLRETYGEMADCCAKQEPERNECFLQHKDDNPNLPRLVRPEVDVMCTAFHDNEETFLKKYLYEIARRHPYFYAPELLFFAKRYKAAFTECCQAADKAACLLPKLDELRDEGKASSAKQRLKCASLQKFGERAFKAWAVARLSQRFPKAEFAEVSKLVTDLTKVHTECCHGDLLECADDRADLAKYICENCDSISSKLKECCEKPLLEKSHCIAEVENDEMPADLPSLAADFVESKDVCKNYAEAKDVFLGMFLYEYARRHPDYSVVLLLRLAKTYETTLEKCCAAADPHECYAKVFDEFKPLVEEPQNLIKQNCELFEQLGEYKFQNALLVRYTKKVPQVSTPTLVEVSRNLGKVGSKCCKHPEAKRMPCAEDYLSVVLNQLCVLHEKTPVSDRVTKCCTESLVNRRPCFSALEVDETYVPKEFNAETFTFHADICTLSEKERQIKKQTALVELVKHKPKATKEQLKAVMDDFAAFVEKCCKADDKETCFAEEGKKLVAASQAALGL

SEQ ID NO: 125 - protein, 585 aa, Artificial Sequence
  HSA C34A_I271C
DAHKSEVAHRFKDLGEENFKALVLIAFAQYLQQAPFEDHVKLVNEVTEFAKTCVADESAENCDKSLHTLFGDKLCTVATLRETYGEMADCCAKQEPERNECFLQHKDDNPNLPRLVRPEVDVMCTAFHDNEETFLKKYLYEIARRHPYFYAPELLFFAKRYKAAFTECCQAADKAACLLPKLDELRDEGKASSAKQRLKCASLQKFGERAFKAWAVARLSQRFPKAEFAEVSKLVTDLTKVHTECCHGDLLECADDRADLAKYICENQDSCSSKLKECCEKPLLEKSHCIAEVENDEMPADLPSLAADFVESKDVCKNYAEAKDVFLGMFLYEYARRHPDYSVVLLLRLAKTYETTLEKCCAAADPHECYAKVFDEFKPLVEEPQNLIKQNCELFEQLGEYKFQNALLVRYTKKVPQVSTPTLVEVSRNLGKVGSKCCKHPEAKRMPCAEDYLSVVLNQLCVLHEKTPVSDRVTKCCTESLVNRRPCFSALEVDETYVPKEFNAETFTFHADICTLSEKERQIKKQTALVELVKHKPKATKEQLKAVMDDFAAFVEKCCKADDKETCFAEEGKKLVAASQAALGL

SEQ ID NO: 126 - protein, 585 aa, Artificial Sequence
  HSA C34A_L275C
DAHKSEVAHRFKDLGEENFKALVLIAFAQYLQQAPFEDHVKLVNEVTEFAKTCVADESAENCDKSLHTLFGDKLCTVATLRETYGEMADCCAKQEPERNECFLQHKDDNPNLPRLVRPEVDVMCTAFHDNEETFLKKYLYEIARRHPYFYAPELLFFAKRYKAAFTECCQAADKAACLLPKLDELRDEGKASSAKQRLKCASLQKFGERAFKAWAVARLSQRFPKAEFAEVSKLVTDLTKVHTECCHGDLLECADDRADLAKYICENQDSISSKCKECCEKPLLEKSHCIAEVENDEMPADLPSLAADFVESKDVCKNYAEAKDVFLGMFLYEYARRHPDYSVVLLLRLAKTYETTLEKCCAAADPHECYAKVFDEFKPLVEEPQNLIKQNCELFEQLGEYKFQNALLVRYTKKVPQVSTPTLVEVSRNLGKVGSKCCKHPEAKRMPCAEDYLSVVLNQLCVLHEKTPVSDRVTKCCTESLVNRRPCFSALEVDETYVPKEFNAETFTFHADICTLSEKERQIKKQTALVELVKHKPKATKEQLKAVMDDFAAFVEKCCKADDKETCFAEEGKKLVAASQAALGL

SEQ ID NO: 127 - protein, 585 aa, Artificial Sequence
  HSA C34A_E277C
DAHKSEVAHRFKDLGEENFKALVLIAFAQYLQQAPFEDHVKLVNEVTEFAKTCVADESAENCDKSLHTLFGDKLCTVATLRETYGEMADCCAKQEPERNECFLQHKDDNPNLPRLVRPEVDVMCTAFHDNEETFLKKYLYEIARRHPYFYAPELLFFAKRYKAAFTECCQAADKAACLLPKLDELRDEGKASSAKQRLKCASLQKFGERAFKAWAVARLSQRFPKAEFAEVSKLVTDLTKVHTECCHGDLLECADDRADLAKYICENQDSISSKLKCCCEKPLLEKSHCIAEVENDEMPADLPSLAADFVESKDVCKNYAEAKDVFLGMFLYEYARRHPDYSVVLLLRLAKTYETTLEKCCAAADPHECYAKVFDEFKPLVEEPQNLIKQNCELFEQLGEYKFQNALLVRYTKKVPQVSTPTLVEVSRNLGKVGSKCCKHPEAKRMPCAEDYLSVVLNQLCVLHEKTPVSDRVTKCCTESLVNRRPCFSALEVDETYVPKEFNAETFTFHADICTLSEKERQIKKQTALVELVKHKPKATKEQLKAVMDDFAAFVEKCCKADDKETCFAEEGKKLVAASQAALGL

SEQ ID NO: 128 - protein, 585 aa, Artificial Sequence
  HSA C34A_L284C
DAHKSEVAHRFKDLGEENFKALVLIAFAQYLQQAPFEDHVKLVNEVTEFAKTCVADESAENCDKSLHTLFGDKLCTVATLRETYGEMADCCAKQEPERNECFLQHKDDNPNLPRLVRPEVDVMCTAFHDNEETFLKKYLYEIARRHPYFYAPELLFFAKRYKAAFTECCQAADKAACLLPKLDELRDEGKASSAKQRLKCASLQKFGERAFKAWAVARLSQRFPKAEFAEVSKLVTDLTKVHTECCHGDLLECADDRADLAKYICENQDSISSKLKECCEKPLCEKSHCIAEVENDEMPADLPSLAADFVESKDVCKNYAEAKDVFLGMFLYEYARRHPDYSVVLLLRLAKTYETTLEKCCAAADPHECYAKVFDEFKPLVEEPQNLIKQNCELFEQLGEYKFQNALLVRYTKKVPQVSTPTLVEVSRNLGKVGSKCCKHPEAKRMPCAEDYLSVVLNQLCVLHEKTPVSDRVTKCCTESLVNRRPCFSALEVDETYVPKEFNAETFTFHADICTLSEKERQIKKQTALVELVKHKPKATKEQLKAVMDDFAAFVEKCCKADDKETCFAEEGKKLVAASQAALGL

SEQ ID NO: 129 - protein, 585 aa, Artificial Sequence
  HSA C34A_E294C
DAHKSEVAHRFKDLGEENFKALVLIAFAQYLQQAPFEDHVKLVNEVTEFAKTCVADESAENCDKSLHTLFGDKLCTVATLRETYGEMADCCAKQEPERNECFLQHKDDNPNLPRLVRPEVDVMCTAFHDNEETFLKKYLYEIARRHPYFYAPELLFFAKRYKAAFTECCQAADKAACLLPKLDELRDEGKASSAKQRLKCASLQKFGERAFKAWAVARLSQRFPKAEFAEVSKLVTDLTKVHTECCHGDLLECADDRADLAKYICENQDSISSKLKECCEKPLLEKSHCIAEVCNDEMPADLPSLAADFVESKDVCKNYAEAKDVFLGMFLYEYARRHPDYSVVLLLRLAKTYETTLEKCCAAADPHECYAKVFDEFKPLVEEPQNLIKQNCELFEQLGEYKFQNALLVRYTKKVPQVSTPTLVEVSRNLGKVGSKCCKHPEAKRMPCAEDYLSVVLNQLCVLHEKTPVSDRVTKCCTESLVNRRPCFSALEVDETYVPKEFNAETFTFHADICTLSEKERQIKKQTALVELVKHKPKATKEQLKAVMDDFAAFVEKCCKADDKETCFAEEGKKLVAASQAALGL

SEQ ID NO: 130 - protein, 585 aa, Artificial Sequence
  HSA C34A_E311C
DAHKSEVAHRFKDLGEENFKALVLIAFAQYLQQAPFEDHVKLVNEVTEFAKTCVADESAENCDKSLHTLFGDKLCTVATLRETYGEMADCCAKQEPERNECFLQHKDDNPNLPRLVRPEVDVMCTAFHDNEETFLKKYLYEIARRHPYFYAPELLFFAKRYKAAFTECCQAADKAACLLPKLDELRDEGKASSAKQRLKCASLQKFGERAFKAWAVARLSQRFPKAEFAEVSKLVTDLTKVHTECCHGDLLECADDRADLAKYICENQDSISSKLKECCEKPLLEKSHCIAEVENDEMPADLPSLAADFVCSKDVCKNYAEAKDVFLGMFLYEYARRHPDYSVVLLLRLAKTYETTLEKCCAAADPHECYAKVFDEFKPLVEEPQNLIKQNCELFEQLGEYKFQNALLVRYTKKVPQVSTPTLVEVSRNLGKVGSKCCKHPEAKRMPCAEDYLSVVLNQLCVLHEKTPVSDRVTKCCTESLVNRRPCFSALEVDETYVPKEFNAETFTFHADICTLSEKERQIKKQTALVELVKHKPKATKEQLKAVMDDFAAFVEKCCKADDKETCFAEEGKKLVAASQAALGL

SEQ ID NO: 131 - protein, 585 aa, Artificial Sequence
  HSA C34A_K317C
DAHKSEVAHRFKDLGEENFKALVLIAFAQYLQQAPFEDHVKLVNEVTEFAKTCVADESAENCDKSLHTLFGDKLCTVATLRETYGEMADCCAKQEPERNECFLQHKDDNPNLPRLVRPEVDVMCTAFHDNEETFLKKYLYEIARRHPYFYAPELLFFAKRYKAAFTECCQAADKAACLLPKLDELRDEGKASSAKQRLKCASLQKFGERAFKAWAVARLSQRFPKAEFAEVSKLVTDLTKVHTECCHGDLLECADDRADLAKYICENQDSISSKLKECCEKPLLEKSHCIAEVENDEMPADLPSLAADFVESKDVCCNYAEAKDVFLGMFLYEYARRHPDYSVVLLLRLAKTYETTLEKCCAAADPHECYAKVFDEFKPLVEEPQNLIKQNCELFEQLGEYKFQNALLVRYTKKVPQVSTPTLVEVSRNLGKVGSKCCKHPEAKRMPCAEDYLSVVLNQLCVLHEKTPVSDRVTKCCTESLVNRRPCFSALEVDETYVPKEFNAETFTFHADICTLSEKERQIKKQTALVELVKHKPKATKEQLKAVMDDFAAFVEKCCKADDKETCFAEEGKKLVAASQAALGL

SEQ ID NO: 132 - protein, 585 aa, Artificial Sequence
  HSA C34A_A322C
DAHKSEVAHRFKDLGEENFKALVLIAFAQYLQQAPFEDHVKLVNEVTEFAKTCVADESAENCDKSLHTLFGDKLCTVATLRETYGEMADCCAKQEPERNECFLQHKDDNPNLPRLVRPEVDVMCTAFHDNEETFLKKYLYEIARRHPYFYAPELLFFAKRYKAAFTECCQAADKAACLLPKLDELRDEGKASSAKQRLKCASLQKFGERAFKAWAVARLSQRFPKAEFAEVSKLVTDLTKVHTECCHGDLLECADDRADLAKYICENQDSISSKLKECCEKPLLEKSHCIAEVENDEMPADLPSLAADFVESKDVCKNYAECKDVFLGMFLYEYARRHPDYSVVLLLRLAKTYETTLEKCCAAADPHECYAKVFDEFKPLVEEPQNLIKQNCELFEQLGEYKFQNALLVRYTKKVPQVSTPTLVEVSRNLGKVGSKCCKHPEAKRMPCAEDYLSVVLNQLCVLHEKTPVSDRVTKCCTESLVNRRPCFSALEVDETYVPKEFNAETFTFHADICTLSEKERQIKKQTALVELVKHKPKATKEQLKAVMDDFAAFVEKCCKADDKETCFAEEGKKLVAASQAALGL

SEQ ID NO: 133 - protein, 585 aa, Artificial Sequence
  HSA C34A_E333C
DAHKSEVAHRFKDLGEENFKALVLIAFAQYLQQAPFEDHVKLVNEVTEFAKTCVADESAENCDKSLHTLFGDKLCTVATLRETYGEMADCCAKQEPERNECFLQHKDDNPNLPRLVRPEVDVMCTAFHDNEETFLKKYLYEIARRHPYFYAPELLFFAKRYKAAFTECCQAADKAACLLPKLDELRDEGKASSAKQRLKCASLQKFGERAFKAWAVARLSQRFPKAEFAEVSKLVTDLTKVHTECCHGDLLECADDRADLAKYICENQDSISSKLKECCEKPLLEKSHCIAEVENDEMPADLPSLAADFVESKDVCKNYAEAKDVFLGMFLYCYARRHPDYSVVLLLRLAKTYETTLEKCCAAADPHECYAKVFDEFKPLVEEPQNLIKQNCELFEQLGEYKFQNALLVRYTKKVPQVSTPTLVEVSRNLGKVGSKCCKHPEAKRMPCAEDYLSVVLNQLCVLHEKTPVSDRVTKCCTESLVNRRPCFSALEVDETYVPKEFNAETFTFHADICTLSEKERQIKKQTALVELVKHKPKATKEQLKAVMDDFAAFVEKCCKADDKETCFAEEGKKLVAASQAALGL

SEQ ID NO: 134 - protein, 585 aa, Artificial Sequence
  HSA C34A_D340C
DAHKSEVAHRFKDLGEENFKALVLIAFAQYLQQAPFEDHVKLVNEVTEFAKTCVADESAENCDKSLHTLFGDKLCTVATLRETYGEMADCCAKQEPERNECFLQHKDDNPNLPRLVRPEVDVMCTAFHDNEETFLKKYLYEIARRHPYFYAPELLFFAKRYKAAFTECCQAADKAACLLPKLDELRDEGKASSAKQRLKCASLQKFGERAFKAWAVARLSQRFPKAEFAEVSKLVTDLTKVHTECCHGDLLECADDRADLAKYICENQDSISSKLKECCEKPLLEKSHCIAEVENDEMPADLPSLAADFVESKDVCKNYAEAKDVFLGMFLYEYARRHPCYSVVLLLRLAKTYETTLEKCCAAADPHECYAKVFDEFKPLVEEPQNLIKQNCELFEQLGEYKFQNALLVRYTKKVPQVSTPTLVEVSRNLGKVGSKCCKHPEAKRMPCAEDYLSVVLNQLCVLHEKTPVSDRVTKCCTESLVNRRPCFSALEVDETYVPKEFNAETFTFHADICTLSEKERQIKKQTALVELVKHKPKATKEQLKAVMDDFAAFVEKCCKADDKETCFAEEGKKLVAASQAALGL

SEQ ID NO: 135 - protein, 585 aa, Artificial Sequence
  HSA C34A_E354C
DAHKSEVAHRFKDLGEENFKALVLIAFAQYLQQAPFEDHVKLVNEVTEFAKTCVADESAENCDKSLHTLFGDKLCTVATLRETYGEMADCCAKQEPERNECFLQHKDDNPNLPRLVRPEVDVMCTAFHDNEETFLKKYLYEIARRHPYFYAPELLFFAKRYKAAFTECCQAADKAACLLPKLDELRDEGKASSAKQRLKCASLQKFGERAFKAWAVARLSQRFPKAEFAEVSKLVTDLTKVHTECCHGDLLECADDRADLAKYICENQDSISSKLKECCEKPLLEKSHCIAEVENDEMPADLPSLAADFVESKDVCKNYAEAKDVFLGMFLYEYARRHPDYSVVLLLRLAKTYCTTLEKCCAAADPHECYAKVFDEFKPLVEEPQNLIKQNCELFEQLGEYKFQNALLVRYTKKVPQVSTPTLVEVSRNLGKVGSKCCKHPEAKRMPCAEDYLSVVLNQLCVLHEKTPVSDRVTKCCTESLVNRRPCFSALEVDETYVPKEFNAETFTFHADICTLSEKERQIKKQTALVELVKHKPKATKEQLKAVMDDFAAFVEKCCKADDKETCFAEEGKKLVAASQAALGL

SEQ ID NO: 136 - protein, 585 aa, Artificial Sequence
  HSA C34A_E358C
DAHKSEVAHRFKDLGEENFKALVLIAFAQYLQQAPFEDHVKLVNEVTEFAKTCVADESAENCDKSLHTLFGDKLCTVATLRETYGEMADCCAKQEPERNECFLQHKDDNPNLPRLVRPEVDVMCTAFHDNEETFLKKYLYEIARRHPYFYAPELLFFAKRYKAAFTECCQAADKAACLLPKLDELRDEGKASSAKQRLKCASLQKFGERAFKAWAVARLSQRFPKAEFAEVSKLVTDLTKVHTECCHGDLLECADDRADLAKYICENQDSISSKLKECCEKPLLEKSHCIAEVENDEMPADLPSLAADFVESKDVCKNYAEAKDVFLGMFLYEYARRHPDYSVVLLLRLAKTYETTLCKCCAAADPHECYAKVFDEFKPLVEEPQNLIKQNCELFEQLGEYKFQNALLVRYTKKVPQVSTPTLVEVSRNLGKVGSKCCKHPEAKRMPCAEDYLSVVLNQLCVLHEKTPVSDRVTKCCTESLVNRRPCFSALEVDETYVPKEFNAETFTFHADICTLSEKERQIKKQTALVELVKHKPKATKEQLKAVMDDFAAFVEKCCKADDKETCFAEEGKKLVAASQAALGL

SEQ ID NO: 137 - protein, 585 aa, Artificial Sequence
  HSA C34A_K359C
DAHKSEVAHRFKDLGEENFKALVLIAFAQYLQQAPFEDHVKLVNEVTEFAKTCVADESAENCDKSLHTLFGDKLCTVATLRETYGEMADCCAKQEPERNECFLQHKDDNPNLPRLVRPEVDVMCTAFHDNEETFLKKYLYEIARRHPYFYAPELLFFAKRYKAAFTECCQAADKAACLLPKLDELRDEGKASSAKQRLKCASLQKFGERAFKAWAVARLSQRFPKAEFAEVSKLVTDLTKVHTECCHGDLLECADDRADLAKYICENQDSISSKLKECCEKPLLEKSHCIAEVENDEMPADLPSLAADFVESKDVCKNYAEAKDVFLGMFLYEYARRHPDYSVVLLLRLAKTYETTLECCCAAADPHECYAKVFDEFKPLVEEPQNLIKQNCELFEQLGEYKFQNALLVRYTKKVPQVSTPTLVEVSRNLGKVGSKCCKHPEAKRMPCAEDYLSVVLNQLCVLHEKTPVSDRVTKCCTESLVNRRPCFSALEVDETYVPKEFNAETFTFHADICTLSEKERQIKKQTALVELVKHKPKATKEQLKAVMDDFAAFVEKCCKADDKETCFAEEGKKLVAASQAALGL

SEQ ID NO: 138 - protein, 585 aa, Artificial Sequence
  HSA C34A_A362C
DAHKSEVAHRFKDLGEENFKALVLIAFAQYLQQAPFEDHVKLVNEVTEFAKTCVADESAENCDKSLHTLFGDKLCTVATLRETYGEMADCCAKQEPERNECFLQHKDDNPNLPRLVRPEVDVMCTAFHDNEETFLKKYLYEIARRHPYFYAPELLFFAKRYKAAFTECCQAADKAACLLPKLDELRDEGKASSAKQRLKCASLQKFGERAFKAWAVARLSQRFPKAEFAEVSKLVTDLTKVHTECCHGDLLECADDRADLAKYICENQDSISSKLKECCEKPLLEKSHCIAEVENDEMPADLPSLAADFVESKDVCKNYAEAKDVFLGMFLYEYARRHPDYSVVLLLRLAKTYETTLEKCCCAADPHECYAKVFDEFKPLVEEPQNLIKQNCELFEQLGEYKFQNALLVRYTKKVPQVSTPTLVEVSRNLGKVGSKCCKHPEAKRMPCAEDYLSVVLNQLCVLHEKTPVSDRVTKCCTESLVNRRPCFSALEVDETYVPKEFNAETFTFHADICTLSEKERQIKKQTALVELVKHKPKATKEQLKAVMDDFAAFVEKCCKADDKETCFAEEGKKLVAASQAALGL

SEQ ID NO: 139 - protein, 585 aa, Artificial Sequence
  HSA C34A_E382C
DAHKSEVAHRFKDLGEENFKALVLIAFAQYLQQAPFEDHVKLVNEVTEFAKTCVADESAENCDKSLHTLFGDKLCTVATLRETYGEMADCCAKQEPERNECFLQHKDDNPNLPRLVRPEVDVMCTAFHDNEETFLKKYLYEIARRHPYFYAPELLFFAKRYKAAFTECCQAADKAACLLPKLDELRDEGKASSAKQRLKCASLQKFGERAFKAWAVARLSQRFPKAEFAEVSKLVTDLTKVHTECCHGDLLECADDRADLAKYICENQDSISSKLKECCEKPLLEKSHCIAEVENDEMPADLPSLAADFVESKDVCKNYAEAKDVFLGMFLYEYARRHPDYSVVLLLRLAKTYETTLEKCCAAADPHECYAKVFDEFKPLVCEPQNLIKQNCELFEQLGEYKFQNALLVRYTKKVPQVSTPTLVEVSRNLGKVGSKCCKHPEAKRMPCAEDYLSVVLNQLCVLHEKTPVSDRVTKCCTESLVNRRPCFSALEVDETYVPKEFNAETFTFHADICTLSEKERQIKKQTALVELVKHKPKATKEQLKAVMDDFAAFVEKCCKADDKETCFAEEGKKLVAASQAALGL

SEQ ID NO: 140 - protein, 585 aa, Artificial Sequence
  HSA C34A_L398C
DAHKSEVAHRFKDLGEENFKALVLIAFAQYLQQAPFEDHVKLVNEVTEFAKTCVADESAENCDKSLHTLFGDKLCTVATLRETYGEMADCCAKQEPERNECFLQHKDDNPNLPRLVRPEVDVMCTAFHDNEETFLKKYLYEIARRHPYFYAPELLFFAKRYKAAFTECCQAADKAACLLPKLDELRDEGKASSAKQRLKCASLQKFGERAFKAWAVARLSQRFPKAEFAEVSKLVTDLTKVHTECCHGDLLECADDRADLAKYICENQDSISSKLKECCEKPLLEKSHCIAEVENDEMPADLPSLAADFVESKDVCKNYAEAKDVFLGMFLYEYARRHPDYSVVLLLRLAKTYETTLEKCCAAADPHECYAKVFDEFKPLVEEPQNLIKQNCELFEQCGEYKFQNALLVRYTKKVPQVSTPTLVEVSRNLGKVGSKCCKHPEAKRMPCAEDYLSVVLNQLCVLHEKTPVSDRVTKCCTESLVNRRPCFSALEVDETYVPKEFNAETFTFHADICTLSEKERQIKKQTALVELVKHKPKATKEQLKAVMDDFAAFVEKCCKADDKETCFAEEGKKLVAASQAALGL

SEQ ID NO: 141 - protein, 585 aa, Artificial Sequence
  HSA C34A_K93C_E294C
DAHKSEVAHRFKDLGEENFKALVLIAFAQYLQQAPFEDHVKLVNEVTEFAKTCVADESAENCDKSLHTLFGDKLCTVATLRETYGEMADCCACQEPERNECFLQHKDDNPNLPRLVRPEVDVMCTAFHDNEETFLKKYLYEIARRHPYFYAPELLFFAKRYKAAFTECCQAADKAACLLPKLDELRDEGKASSAKQRLKCASLQKFGERAFKAWAVARLSQRFPKAEFAEVSKLVTDLTKVHTECCHGDLLECADDRADLAKYICENQDSISSKLKECCEKPLLEKSHCIAEVCNDEMPADLPSLAADFVESKDVCKNYAEAKDVFLGMFLYEYARRHPDYSVVLLLRLAKTYETTLEKCCAAADPHECYAKVFDEFKPLVEEPQNLIKQNCELFEQLGEYKFQNALLVRYTKKVPQVSTPTLVEVSRNLGKVGSKCCKHPEAKRMPCAEDYLSVVLNQLCVLHEKTPVSDRVTKCCTESLVNRRPCFSALEVDETYVPKEFNAETFTFHADICTLSEKERQIKKQTALVELVKHKPKATKEQLKAVMDDFAAFVEKCCKADDKETCFAEEGKKLVAASQAALGL

SEQ ID NO: 142 - protein, 585 aa, Artificial Sequence [sequence omitted]

SEQ ID NO: 143 - protein, 585 aa, Artificial Sequence [sequence omitted]

SEQ ID NO: 144 - protein, 585 aa, Artificial Sequence
  HSA K93C_E294C
DAHKSEVAHRFKDLGEENFKALVLIAFAQYLQQCPFEDHVKLVNEVTEFAKTCVADESAENCDKSLHTLFGDKLCTVATLRETYGEMADCCACQEPERNECFLQHKDDNPNLPRLVRPEVDVMCTAFHDNEETFLKKYLYEIARRHPYFYAPELLFFAKRYKAAFTECCQAADKAACLLPKLDELRDEGKASSAKQRLKCASLQKFGERAFKAWAVARLSQRFPKAEFAEVSKLVTDLTKVHTECCHGDLLECADDRADLAKYICENQDSISSKLKECCEKPLLEKSHCIAEVCNDEMPADLPSLAADFVESKDVCKNYAEAKDVFLGMFLYEYARRHPDYSVVLLLRLAKTYETTLEKCCAAADPHECYAKVFDEFKPLVEEPQNLIKQNCELFEQLGEYKFQNALLVRYTKKVPQVSTPTLVEVSRNLGKVGSKCCKHPEAKRMPCAEDYLSVVLNQLCVLHEKTPVSDRVTKCCTESLVNRRPCFSALEVDETYVPKEFNAETFTFHADICTLSEKERQIKKQTALVELVKHKPKATKEQLKAVMDDFAAFVEKCCKADDKETCFAEEGKKLVAASQAALGL

SEQ ID NO: 145 - protein, 585 aa, Artificial Sequence
  HSA K573P
DAHKSEVAHRFKDLGEENFKALVLIAFAQYLQQCPFEDHVKLVNEVTEFAKTCVADESAENCDKSLHTLFGDKLCTVATLRETYGEMADCCAKQEPERNECFLQHKDDNPNLPRLVRPEVDVMCTAFHDNEETFLKKYLYEIARRHPYFYAPELLFFAKRYKAAFTECCQAADKAACLLPKLDELRDEGKASSAKQRLKCASLQKFGERAFKAWAVARLSQRFPKAEFAEVSKLVTDLTKVHTECCHGDLLECADDRADLAKYICENQDSISSKLKECCEKPLLEKSHCIAEVENDEMPADLPSLAADFVESKDVCKNYAEAKDVFLGMFLYEYARRHPDYSVVLLLRLAKTYETTLEKCCAAADPHECYAKVFDEFKPLVEEPQNLIKQNCELFEQLGEYKFQNALLVRYTKKVPQVSTPTLVEVSRNLGKVGSKCCKHPEAKRMPCAEDYLSVVLNQLCVLHEKTPVSDRVTKCCTESLVNRRPCFSALEVDETYVPKEFNAETFTFHADICTLSEKERQIKKQTALVELVKHKPKATKEQLKAVMDDFAAFVEKCCKADDKETCFAEEGPKLVAASQAALGL

SEQ ID NO: 146 - protein, 585 aa, Artificial Sequence
  HSA C34A_K93C_K573P
DAHKSEVAHRFKDLGEENFKALVLIAFAQYLQQAPFEDHVKLVNEVTEFAKTCVADESAENCDKSLHTLFGDKLCTVATLRETYGEMADCCACQEPERNECFLQHKDDNPNLPRLVRPEVDVMCTAFHDNEETFLKKYLYEIARRHPYFYAPELLFFAKRYKAAFTECCQAADKAACLLPKLDELRDEGKASSAKQRLKCASLQKFGERAFKAWAVARLSQRFPKAEFAEVSKLVTDLTKVHTECCHGDLLECADDRADLAKYICENQDSISSKLKECCEKPLLEKSHCIAEVENDEMPADLPSLAADFVESKDVCKNYAEAKDVFLGMFLYEYARRHPDYSVVLLLRLAKTYETTLEKCCAAADPHECYAKVFDEFKPLVEEPQNLIKQNCELFEQLGEYKFQNALLVRYTKKVPQVSTPTLVEVSRNLGKVGSKCCKHPEAKRMPCAEDYLSVVLNQLCVLHEKTPVSDRVTKCCTESLVNRRPCFSALEVDETYVPKEFNAETFTFHADICTLSEKERQIKKQTALVELVKHKPKATKEQLKAVMDDFAAFVEKCCKADDKETCFAEEGPKLVAASQAALGL

SEQ ID NO: 147 - protein, 585 aa, Artificial Sequence
  HSA C34A_E294C_K573P
DAHKSEVAHRFKDLGEENFKALVLIAFAQYLQQAPFEDHVKLVNEVTEFAKTCVADESAENCDKSLHTLFGDKLCTVATLRETYGEMADCCAKQEPERNECFLQHKDDNPNLPRLVRPEVDVMCTAFHDNEETFLKKYLYEIARRHPYFYAPELLFFAKRYKAAFTECCQAADKAACLLPKLDELRDEGKASSAKQRLKCASLQKFGERAFKAWAVARLSQRFPKAEFAEVSKLVTDLTKVHTECCHGDLLECADDRADLAKYICENQDSISSKLKECCEKPLLEKSHCIAEVCNDEMPADLPSLAADFVESKDVCKNYAEAKDVFLGMFLYEYARRHPDYSVVLLLRLAKTYETTLEKCCAAADPHECYAKVFDEFKPLVEEPQNLIKQNCELFEQLGEYKFQNALLVRYTKKVPQVSTPTLVEVSRNLGKVGSKCCKHPEAKRMPCAEDYLSVVLNQLCVLHEKTPVSDRVTKCCTESLVNRRPCFSALEVDETYVPKEFNAETFTFHADICTLSEKERQIKKQTALVELVKHKPKATKEQLKAVMDDFAAFVEKCCKADDKETCFAEEGPKLVAASQAALGL

SEQ ID NO: 148 - protein, 585 aa, Artificial Sequence [sequence omitted]

SEQ ID NO: 149 - protein, 585 aa, Artificial Sequence
  HSA K93C_K573P
DAHKSEVAHRFKDLGEENFKALVLIAFAQYLQQCPFEDHVKLVNEVTEFAKTCVADESAENCDKSLHTLFGDKLCTVATLRETYGEMADCCACQEPERNECFLQHKDDNPNLPRLVRPEVDVMCTAFHDNEETFLKKYLYEIARRHPYFYAPELLFFAKRYKAAFTECCQAADKAACLLPKLDELRDEGKASSAKQRLKCASLQKFGERAFKAWAVARLSQRFPKAEFAEVSKLVTDLTKVHTECCHGDLLECADDRADLAKYICENQDSISSKLKECCEKPLLEKSHCIAEVENDEMPADLPSLAADFVESKDVCKNYAEAKDVFLGMFLYEYARRHPDYSVVLLLRLAKTYETTLEKCCAAADPHECYAKVFDEFKPLVEEPQNLIKQNCELFEQLGEYKFQNALLVRYTKKVPQVSTPTLVEVSRNLGKVGSKCCKHPEAKRMPCAEDYLSVVLNQLCVLHEKTPVSDRVTKCCTESLVNRRPCFSALEVDETYVPKEFNAETFTFHADICTLSEKERQIKKQTALVELVKHKPKATKEQLKAVMDDFAAFVEKCCKADDKETCFAEEGPKLVAASQAALGL

SEQ ID NO: 150 - protein, 585 aa, Artificial Sequence
  HSA E294C_K573P
DAHKSEVAHRFKDLGEENFKALVLIAFAQYLQQCPFEDHVKLVNEVTEFAKTCVADESAENCDKSLHTLFGDKLCTVATLRETYGEMADCCAKQEPERNECFLQHKDDNPNLPRLVRPEVDVMCTAFHDNEETFLKKYLYEIARRHPYFYAPELLFFAKRYKAAFTECCQAADKAACLLPKLDELRDEGKASSAKQRLKCASLQKFGERAFKAWAVARLSQRFPKAEFAEVSKLVTDLTKVHTECCHGDLLECADDRADLAKYICENQDSISSKLKECCEKPLLEKSHCIAEVCNDEMPADLPSLAADFVESKDVCKNYAEAKDVFLGMFLYEYARRHPDYSVVLLLRLAKTYETTLEKCCAAADPHECYAKVFDEFKPLVEEPQNLIKQNCELFEQLGEYKFQNALLVRYTKKVPQVSTPTLVEVSRNLGKVGSKCCKHPEAKRMPCAEDYLSVVLNQLCVLHEKTPVSDRVTKCCTESLVNRRPCFSALEVDETYVPKEFNAETFTFHADICTLSEKERQIKKQTALVELVKHKPKATKEQLKAVMDDFAAFVEKCCKADDKETCFAEEGPKLVAASQAALGL

SEQ ID NO: 151 - protein, 585 aa, Artificial Sequence
  HSA K93C_E294C_K573P
DAHKSEVAHRFKDLGEENFKALVLIAFAQYLQQCPFEDHVKLVNEVTEFAKTCVADESAENCDKSLHTLFGDKLCTVATLRETYGEMADCCACQEPERNECFLQHKDDNPNLPRLVRPEVDVMCTAFHDNEETFLKKYLYEIARRHPYFYAPELLFFAKRYKAAFTECCQAADKAACLLPKLDELRDEGKASSAKQRLKCASLQKFGERAFKAWAVARLSQRFPKAEFAEVSKLVTDLTKVHTECCHGDLLECADDRADLAKYICENQDSISSKLKECCEKPLLEKSHCIAEVCNDEMPADLPSLAADFVESKDVCKNYAEAKDVFLGMFLYEYARRHPDYSVVLLLRLAKTYETTLEKCCAAADPHECYAKVFDEFKPLVEEPQNLIKQNCELFEQLGEYKFQNALLVRYTKKVPQVSTPTLVEVSRNLGKVGSKCCKHPEAKRMPCAEDYLSVVLNQLCVLHEKTPVSDRVTKCCTESLVNRRPCFSALEVDETYVPKEFNAETFTFHADICTLSEKERQIKKQTALVELVKHKPKATKEQLKAVMDDFAAFVEKCCKADDKETCFAEEGPKLVAASQAALGL

SEQ ID NO: 152 - protein, 585 aa, Artificial Sequence
  HSA C34A_L302C
DAHKSEVAHRFKDLGEENFKALVLIAFAQYLQQAPFEDHVKLVNEVTEFAKTCVADESAENCDKSLHTLFGDKLCTVATLRETYGEMADCCAKQEPERNECFLQHKDDNPNLPRLVRPEVDVMCTAFHDNEETFLKKYLYEIARRHPYFYAPELLFFAKRYKAAFTECCQAADKAACLLPKLDELRDEGKASSAKQRLKCASLQKFGERAFKAWAVARLSQRFPKAEFAEVSKLVTDLTKVHTECCHGDLLECADDRADLAKYICENQDSISSKLKECCEKPLLEKSHCIAEVENDEMPADCPSLAADFVESKDVCKNYAEAKDVFLGMFLYEYARRHPDYSVVLLLRLAKTYETTLEKCCAAADPHECYAKVFDEFKPLVEEPQNLIKQNCELFEQLGEYKFQNALLVRYTKKVPQVSTPTLVEVSRNLGKVGSKCCKHPEAKRMPCAEDYLSVVLNQLCVLHEKTPVSDRVTKCCTESLVNRRPCFSALEVDETYVPKEFNAETFTFHADICTLSEKERQIKKQTALVELVKHKPKATKEQLKAVMDDFAAFVEKCCKADDKETCFAEEGKKLVAASQAALGL